European Patent Application EP 4 613 762 A1, published September 10, 2025. Title: KRAS_G12V MUTANT ANTIGEN-SPECIFIC TCR AND REDIRECTED CD4 T CELL CO-EXPRESSING SAME AND CD8. Applicant: Neowise Biotechnology Co., Ltd. Application US. The sequence listing filed with the application follows.

SEQUENCE LISTING (405 sequences)

SEQ ID NO: 1 - protein, 7 aa, synthetic construct
TRDTTYY

SEQ ID NO: 2 - protein, 8 aa, synthetic construct
RNSFDEQN

SEQ ID NO: 3 - protein, 11 aa, synthetic construct
ARDQTGANNLF

SEQ ID NO: 4 - protein, 7 aa, synthetic construct
TRDTTYY

SEQ ID NO: 5 - protein, 8 aa, synthetic construct
RNSFDEQN

SEQ ID NO: 6 - protein, 16 aa, synthetic construct
ALSDPRYSGGGADGLT

SEQ ID NO: 7 - protein, 6 aa, synthetic construct
NSMFDY

SEQ ID NO: 8 - protein, 7 aa, synthetic construct
ISSIKDK

SEQ ID NO: 9 - protein, 10 aa, synthetic construct
AGYQGGYKLS

SEQ ID NO: 10 - protein, 6 aa, synthetic construct
DRGSQS

SEQ ID NO: 11 - protein, 6 aa, synthetic construct
IYSNGD

SEQ ID NO: 12 - protein, 10 aa, synthetic construct
AVNMPGNMLT

SEQ ID NO: 13 - protein, 6 aa, synthetic construct
DSSSTY

SEQ ID NO: 14 - protein, 7 aa, synthetic construct
IFSNMDM

SEQ ID NO: 15 - protein, 12 aa, synthetic construct
AERGTDSWGKLQ

SEQ ID NO: 16 - protein, 5 aa, synthetic construct
TSINN

SEQ ID NO: 17 - protein, 7 aa, synthetic construct
IRSNERE

SEQ ID NO: 18 - protein, 13 aa, synthetic construct
ATDDYGGATNKLI

SEQ ID NO: 19 - protein, 5 aa, synthetic construct
TTSDR

SEQ ID NO: 20 - protein, 7 aa, synthetic construct
LLSNGAV

SEQ ID NO: 21 - protein, 11 aa, synthetic construct
AVDKAAGNKLT

SEQ ID NO: 22 - protein, 6 aa, synthetic construct
VSNAYN

SEQ ID NO: 23 - protein, 4 aa, synthetic construct
GSKP

SEQ ID NO: 24 - protein, 9 aa, synthetic construct
AGSNDYKLS

SEQ ID NO: 25 - protein, 5 aa, synthetic construct
TSINN

SEQ ID NO: 26 - protein, 7 aa, synthetic construct
IRSNERE

SEQ ID NO: 27 - protein, 12 aa, synthetic construct
ATDGGGGADGLT

SEQ ID NO: 28 - protein, 5 aa, synthetic construct
TSINN

SEQ ID NO: 29 - protein, 7 aa, synthetic construct
IRSNERE

SEQ ID NO: 30 - protein, 12 aa, synthetic construct
ATDSGGGADGLT

SEQ ID NO: 31 - protein, 6 aa, synthetic construct
NSMFDY

SEQ ID NO: 32 - protein, 7 aa, synthetic construct
ISSIKDK

SEQ ID NO: 33 - protein, 12 aa, synthetic construct
AASYAGSARQLT

SEQ ID NO: 34 - protein, 6 aa, synthetic construct
DRGSQS

SEQ ID NO: 35 - protein, 6 aa, synthetic construct
IYSNGD

SEQ ID NO: 36 - protein, 11 aa, synthetic construct
ARKKTSYDKVI

SEQ ID NO: 37 - protein, 6 aa, synthetic construct
ATGYPS

SEQ ID NO: 38 - protein, 7 aa, synthetic construct
ATKADDK

SEQ ID NO: 39 - protein, 12 aa, synthetic construct
ALPAGGGADGLT

SEQ ID NO: 40 - protein, 5 aa, synthetic construct
TSINN

SEQ ID NO: 41 - protein, 7 aa, synthetic construct
IRSNERE

SEQ ID NO: 42 - protein, 12 aa, synthetic construct
ATDRTGGYNKLI

SEQ ID NO: 43 - protein, 6 aa, synthetic construct
SSNFYA

SEQ ID NO: 44 - protein, 7 aa, synthetic construct
MTLNGDE

SEQ ID NO: 45 - protein, 10 aa, synthetic construct
AFNNQGGKLI

SEQ ID NO: 46 - protein, 6 aa, synthetic construct
SSYSPS

SEQ ID NO: 47 - protein, 8 aa, synthetic construct
YTSAATLV

SEQ ID NO: 48 - protein, 10 aa, synthetic construct
VVSVWTDKLI

SEQ ID NO: 49 - protein, 92 aa, synthetic construct
AQKVTQAQTEISVVEKEDVTLDCVYETRDTTYYLFWYKQPPSGELVFLIRRNSFDEQNEISGRYSWNFQKSTSSFNFTITASQVVDSAVYFC

SEQ ID NO: 50 - DNA, 276 bp, synthetic construct
  source 1..276: mol_type = other DNA
gctcagaaggtaactcaagcgcagactgaaatttctgtggtggagaaggaggatgtgaccttggactgtgtgtatgaaacccgtgatactacttattacttattctggtacaagcaaccaccaagtggagaattggttttccttattcgtcggaactcttttgatgagcaaaatgaaataagtggtcggtattcttggaacttccagaaatccaccagttccttcaacttcaccatcacagcctcacaagtcgtggactcagcagtatacttctgt

SEQ ID NO: 51 - protein, 19 aa, synthetic construct
QTGANNLFFGTGTRLTVIP

SEQ ID NO: 52 - DNA, 57 bp, synthetic construct
  source 1..57: mol_type = other DNA
caaactggggcaaacaacctcttctttgggactggaacgagactcaccgttattccc

SEQ ID NO: 53 - protein, 95 aa, synthetic construct
AQKVTQAQTEISVVEKEDVTLDCVYETRDTTYYLFWYKQPPSGELVFLIRRNSFDEQNEISGRYSWNFQKSTSSFNFTITASQVVDSAVYFCALS

SEQ ID NO: 54 - DNA, 285 bp, synthetic construct
  source 1..285: mol_type = other DNA
gctcagaaggtaactcaagcgcagactgaaatttctgtggtggagaaggaggatgtgaccttggactgtgtgtatgaaacccgtgatactacttattacttattctggtacaagcaaccaccaagtggagaattggttttccttattcgtcggaactcttttgatgagcaaaatgaaataagtggtcggtattcttggaacttccagaaatccaccagttccttcaacttcaccatcacagcctcacaagtcgtggactcagcagtatacttctgtgctctgagt

SEQ ID NO: 55 - protein, 21 aa, synthetic construct
YSGGGADGLTFGKGTHLIIQP

SEQ ID NO: 56 - DNA, 63 bp, synthetic construct
  source 1..63: mol_type = other DNA
tattcaggaggaggtgctgacggactcacctttggcaaagggactcatctaatcatccagccc

SEQ ID NO: 57 - protein, 91 aa, synthetic construct
DQQVKQNSPSLSVQEGRISILNCDYTNSMFDYFLWYKKYPAEGPTFLISISSIKDKNEDGRFTVFLNKSAKHLSLHIVPSQPGDSAVYFCA

SEQ ID NO: 58 - DNA, 273 bp, synthetic construct
  source 1..273: mol_type = other DNA
gaccagcaagttaagcaaaattcaccatccctgagcgtccaggaaggaagaatttctattctgaactgtgactatactaacagcatgtttgattatttcctatggtacaaaaaataccctgctgaaggtcctacattcctgatatctataagttccattaaggataaaaatgaagatggaagattcactgtcttcttaaacaaaagtgccaagcacctctctctgcacattgtgccctcccagcctggagactctgcagtgtacttctgtgca

SEQ ID NO: 59 - protein, 15 aa, synthetic construct
YKLSFGAGTTVTVRA

SEQ ID NO: 60 - DNA, 45 bp, synthetic construct
  source 1..45: mol_type = other DNA
tacaagctcagctttggagccggaaccacagtaactgtaagagca

SEQ ID NO: 61 - protein, 92 aa, synthetic construct
QKEVEQNSGPLSVPEGAIASLNCTYSDRGSQSFFWYRQYSGKSPELIMFIYSNGDKEDGRFTAQLNKASQYVSLLIRDSQPSDSATYLCAVN

SEQ ID NO: 62 - DNA, 276 bp, synthetic construct
  source 1..276: mol_type = other DNA
cagaaggaggtggagcagaattctggacccctcagtgttccagagggagccattgcctctctcaactgcacttacagtgaccgaggttcccagtccttcttctggtacagacaatattctgggaaaagccctgagttgataatgttcatatactccaatggtgacaaagaagatggaaggtttacagcacagctcaataaagccagccagtatgtttctctgctcatcagagactcccagcccagtgattcagccacctacctctgtgccgtgaac

SEQ ID NO: 63 - protein, 16 aa, synthetic construct
GNMLTFGGGTRLMVKP

SEQ ID NO: 64 - DNA, 48 bp, synthetic construct
  source 1..48: mol_type = other DNA
ggcaacatgctcacctttggagggggaacaaggttaatggtcaaaccc

SEQ ID NO: 65 - protein, 91 aa, synthetic construct
GEDVEQSLFLSVREGDSSVINCTYTDSSSTYLYWYKQEPGAGLQLLTYIFSNMDMKQDQRLTVLLNKKDKHLSLRIADTQTGDSAIYFCAE

SEQ ID NO: 66 - DNA, 273 bp, synthetic construct
  source 1..273: mol_type = other DNA
ggagaggatgtggagcagagtcttttcctgagtgtccgagagggagacagctccgttataaactgcacttacacagacagctcctccacctacttatactggtataagcaagaacctggagcaggtctccagttgctgacgtatattttttcaaatatggacatgaaacaagaccaaagactcactgttctattgaataaaaaggataaacatctgtctctgcgcattgcagacacccagactggggactcagctatctacttctgtgcagag

SEQ ID NO: 67 - protein, 19 aa, synthetic construct
TDSWGKLQFGAGTQVVVTP

SEQ ID NO: 68 - DNA, 57 bp, synthetic construct
  source 1..57: mol_type = other DNA
actgacagctgggggaaattgcagtttggagcagggacccaggttgtggtcacccca

SEQ ID NO: 69 - protein, 92 aa, synthetic construct
SQQGEEDPQALSIQEGENATMNCSYKTSINNLQWYRQNSGRGLVHLILIRSNEREKHSGRLRVTLDTSKKSSSLLITASRAADTASYFCATD

SEQ ID NO: 70 - DNA, 276 bp, synthetic construct
  source 1..276: mol_type = other DNA
agtcaacagggagaagaggatcctcaggccttgagcatccaggagggtgaaaatgccaccatgaactgcagttacaaaactagtataaacaatttacagtggtatagacaaaattcaggtagaggccttgtccacctaattttaatacgttcaaatgaaagagagaaacacagtggaagattaagagtcacgcttgacacttccaagaaaagcagttccttgttgatcacggcttcccgggcagcagacactgcttcttacttctgtgctacggac

SEQ ID NO: 71 - protein, 20 aa, synthetic construct
YGGATNKLIFGTGTLLAVQP

SEQ ID NO: 72 - DNA, 60 bp, synthetic construct
  source 1..60: mol_type = other DNA
tatggtggtgctacaaacaagctcatctttggaactggcactctgcttgctgtccagcca

SEQ ID NO: 73 - protein, 92 aa, synthetic construct
ELKVEQNPLFLSMQEGKNYTIYCNYSTTSDRLYWYRQDPGKSLESLFVLLSNGAVKQEGRLMASLDTKARLSTLHITAAVHDLSATYFCAVD

SEQ ID NO: 74 - DNA, 276 bp, synthetic construct
  source 1..276: mol_type = other DNA
gagctgaaagtggaacaaaaccctctgttcctgagcatgcaggagggaaaaaactataccatctactgcaattattcaaccacttcagacagactgtattggtacaggcaggatcctgggaaaagtctggaatctctgtttgtgttgctatcaaatggagcagtgaagcaggagggacgattaatggcctcacttgataccaaagcccgtctcagcaccctccacatcacagctgccgtgcatgacctctctgccacctacttctgtgccgtggac

SEQ ID NO: 75 - protein, 18 aa, synthetic construct
AAGNKLTFGGGTRVLVKP

SEQ ID NO: 76 - DNA, 54 bp, synthetic construct
  source 1..54: mol_type = other DNA
gctgcaggcaacaagctaacttttggaggaggaaccagggtgctagttaaacca

SEQ ID NO: 77 - protein, 85 aa, synthetic construct
KDQVFQPSTVASSEGAVVEIFCNHSVSNAYNFFWYLHFPGCAPRLLVKGSKPSQQGRYNMTYERFSSSLLILQVREADAAVYYCA

SEQ ID NO: 78 - DNA, 255 bp, synthetic construct
  source 1..255: mol_type = other DNA
aaggaccaagtgtttcagccttccacagtggcatcttcagagggagctgtggtggaaatcttctgtaatcactctgtgtccaatgcttacaacttcttctggtaccttcacttcccgggatgtgcaccaagactccttgttaaaggctcaaagccttctcagcagggacgatacaacatgacctatgaacggttctcttcatcgctgctcatcctccaggtgcgggaggcagatgctgctgtttactactgtgct

SEQ ID NO: 79 - protein, 18 aa, synthetic construct
SNDYKLSFGAGTTVTVRA

SEQ ID NO: 80 - DNA, 54 bp, synthetic construct
  source 1..54: mol_type = other DNA
tctaacgactacaagctcagctttggagccggaaccacagtaactgtaagagca

SEQ ID NO: 81 - protein, 92 aa, synthetic construct; identical to SEQ ID NO: 69

SEQ ID NO: 82 - DNA, 276 bp, synthetic construct; identical to SEQ ID NO: 70
  source 1..276: mol_type = other DNA

SEQ ID NO: 83 - protein, 19 aa, synthetic construct
GGGADGLTFGKGTHLIIQP

SEQ ID NO: 84 - DNA, 57 bp, synthetic construct
  source 1..57: mol_type = other DNA
ggaggaggtgctgacggactcacctttggcaaagggactcatctaatcatccagccc

SEQ ID NO: 85 - protein, 91 aa, synthetic construct
SQQGEEDPQALSIQEGENATMNCSYKTSINNLQWYRQNSGRGLVHLILIRSNEREKHSGRLRVTLDTSKKSSSLLITASRAADTASYFCAT

SEQ ID NO: 86 - DNA, 273 bp, synthetic construct
  source 1..273: mol_type = other DNA
agtcaacagggagaagaggatcctcaggccttgagcatccaggagggtgaaaatgccaccatgaactgcagttacaaaactagtataaacaatttacagtggtatagacaaaattcaggtagaggccttgtccacctaattttaatacgttcaaatgaaagagagaaacacagtggaagattaagagtcacgcttgacacttccaagaaaagcagttccttgttgatcacggcttcccgggcagcagacactgcttcttacttctgtgctacg

SEQ ID NO: 87 - protein, 20 aa, synthetic construct
SGGGADGLTFGKGTHLIIQP

SEQ ID NO: 88 - DNA, 60 bp, synthetic construct
  source 1..60: mol_type = other DNA
tcaggaggaggtgctgacggactcacctttggcaaagggactcatctaatcatccagccc

SEQ ID NO: 89 - protein, 93 aa, synthetic construct
DQQVKQNSPSLSVQEGRISILNCDYTNSMFDYFLWYKKYPAEGPTFLISISSIKDKNEDGRFTVFLNKSAKHLSLHIVPSQPGDSAVYFCAAS

SEQ ID NO: 90 - DNA, 279 bp, synthetic construct
  source 1..279: mol_type = other DNA
gaccagcaagttaagcaaaattcaccatccctgagcgtccaggaaggaagaatttctattctgaactgtgactatactaacagcatgtttgattatttcctatggtacaaaaaataccctgctgaaggtcctacattcctgatatctataagttccattaaggataaaaatgaagatggaagattcactgtcttcttaaacaaaagtgccaagcacctctctctgcacattgtgccctcccagcctggagactctgcagtgtacttctgtgcagcaagc

SEQ ID NO: 91 - protein, 18 aa, synthetic construct
GSARQLTFGSGTQLTVLP

SEQ ID NO: 92 - DNA, 54 bp, synthetic construct
  source 1..54: mol_type = other DNA
ggttctgcaaggcaactgacctttggatctgggacacaattgactgttttacct

SEQ ID NO: 93 - protein, 90 aa, synthetic construct
QKEVEQNSGPLSVPEGAIASLNCTYSDRGSQSFFWYRQYSGKSPELIMFIYSNGDKEDGRFTAQLNKASQYVSLLIRDSQPSDSATYLCA

SEQ ID NO: 94 - DNA, 270 bp, synthetic construct
  source 1..270: mol_type = other DNA
cagaaggaggtggagcagaattctggacccctcagtgttccagagggagccattgcctctctcaactgcacttacagtgaccgaggttcccagtccttcttctggtacagacaatattctgggaaaagccctgagttgataatgttcatatactccaatggtgacaaagaagatggaaggtttacagcacagctcaataaagccagccagtatgtttctctgctcatcagagactcccagcccagtgattcagccacctacctctgtgcc

SEQ ID NO: 95 - protein, 19 aa, synthetic construct
KTSYDKVIFGPGTSLSVIP

SEQ ID NO: 96 - DNA, 57 bp, synthetic construct
  source 1..57: mol_type = other DNA
aaaacctcctacgacaaggtgatatttgggccagggacaagcttatcagtcattcca

SEQ ID NO: 97 - protein, 92 aa, synthetic construct
GNSVTQMEGPVTLSEEAFLTINCTYTATGYPSLFWYVQYPGEGLQLLLKATKADDKGSNKGFEATYRKETTSFHLEKGSVQVSDSAVYFCAL

SEQ ID NO: 98 - DNA, 276 bp, synthetic construct
  source 1..276: mol_type = other DNA
ggaaattcagtgacccagatggaagggccagtgactctctcagaagaggccttcctgactataaactgcacgtacacagccacaggatacccttcccttttctggtatgtccaatatcctggagaaggtctacagctcctcctgaaagccacgaaggctgatgacaagggaagcaacaaaggttttgaagccacataccgtaaagaaaccacttctttccacttggagaaaggctcagttcaagtgtcagactcagcggtgtacttctgtgctctg

SEQ ID NO: 99 - protein, 19 aa, synthetic construct
GGGADGLTFGKGTHLIIQP

SEQ ID NO: 100 - DNA, 57 bp, synthetic construct; identical to SEQ ID NO: 84
  source 1..57: mol_type = other DNA

SEQ ID NO: 101 - protein, 92 aa, synthetic construct; identical to SEQ ID NO: 69

SEQ ID NO: 102 - DNA, 276 bp, synthetic construct; identical to SEQ ID NO: 70
  source 1..276: mol_type = other DNA

SEQ ID NO: 103 - protein, 18 aa, synthetic construct
GGYNKLIFGAGTRLAVHP

SEQ ID NO: 104 - DNA, 54 bp, synthetic construct
  source 1..54: mol_type = other DNA
ggtggctacaataagctgatttttggagcagggaccaggctggctgtacaccca

SEQ ID NO: 105 - protein, 92 aa, synthetic construct
ILNVEQSPQSLHVQEGDSTNFTCSFPSSNFYALHWYRWETAKSPEALFVMTLNGDEKKKGRISATLNTKEGYSYLYIKGSQPEDSATYLCAF

SEQ ID NO: 106 - DNA, 276 bp, synthetic construct
  source 1..276: mol_type = other DNA
atactgaacgtggaacaaagtcctcagtcactgcatgttcaggagggagacagcaccaatttcacctgcagcttcccttccagcaatttttatgccttacactggtacagatgggaaactgcaaaaagccccgaggccttgtttgtaatgactttaaatggggatgaaaagaagaaaggacgaataagtgccactcttaataccaaggagggttacagctatttgtacatcaaaggatcccagcctgaagactcagccacatacctctgtgccttt

SEQ ID NO: 107 - protein, 18 aa, synthetic construct
NQGGKLIFGQGTELSVKP

SEQ ID NO: 108 - DNA, 54 bp, synthetic construct
  source 1..54: mol_type = other DNA
aaccagggaggaaagcttatcttcggacagggaacggagttatctgtgaaaccc

SEQ ID NO: 109 - protein, 94 aa, synthetic construct
AQSVTQLDSHVSVSEGTPVLLRCNYSSSYSPSLFWYVQHPNKGLQLLLKYTSAATLVKGINGFEAEFKKSETSFHLTKPSAHMSDAAEYFCVVS

SEQ ID NO: 110 - DNA, 282 bp, synthetic construct
  source 1..282: mol_type = other DNA
gcccagtcggtgacccagcttgacagccacgtctctgtctctgaaggaaccccggtgctgctgaggtgcaactactcatcttcttattcaccatctctcttctggtatgtgcaacaccccaacaaaggactccagcttctcctgaagtacacatcagcggccaccctggttaaaggcatcaacggttttgaggctgaatttaagaagagtgaaacctccttccacctgacgaaaccctcagcccatatgagcgacgcggctgagtacttctgtgttgtgagt

SEQ ID NO: 111 - protein, 16 aa, synthetic construct
TDKLIFGTGTRLQVFP

SEQ ID NO: 112 - DNA, 48 bp, synthetic construct
  source 1..48: mol_type = other DNA
accgacaagctcatctttgggactgggaccagattacaagtctttcca

SEQ ID NO: 113 - protein, 141 aa, synthetic construct
YIQNPDPAVYQLRDSKSSDKSVCLFTDFDSQTNVSQSKDSDVYITDKTVLDMRSMDFKSNSAVAWSNKSDFACANAFNNSIIPEDTFFPSPESSCDVKLVEKSFETDTNLNFQNLSVIGFRILLLKVAGFNLLMTLRLWSS

SEQ ID NO: 114 - DNA, 423 bp, synthetic construct
  source 1..423: mol_type = other DNA
tatatccagaaccctgaccctgccgtgtaccagctgagagactctaaatccagtgacaagtctgtctgcctattcaccgattttgattctcaaacaaatgtgtcacaaagtaaggattctgatgtgtatatcacagacaaaactgtgctagacatgaggtctatggacttcaagagcaacagtgctgtggcctggagcaacaaatctgactttgcatgtgcaaacgccttcaacaacagcattattccagaagacaccttcttccccagcccagaaagttcctgtgatgtcaagctggtcgagaaaagctttgaaacagatacgaacctaaactttcaaaacctgtcagtgattgggttccgaatcctcctcctgaaagtggccgggtttaatctgctcatgacgctgcggctgtggtccagc

SEQ ID NO: 115 - protein, 141 aa, synthetic construct; identical to SEQ ID NO: 113

SEQ ID NO: 116 - DNA, 423 bp, synthetic construct; identical to SEQ ID NO: 114
  source 1..423: mol_type = other DNA

SEQ ID NO: 117 - protein, 141 aa, synthetic construct
NIQNPDPAVYQLRDSKSSDKSVCLFTDFDSQTNVSQSKDSDVYITDKTVLDMRSMDFKSNSAVAWSNKSDFACANAFNNSIIPEDTFFPSPESSCDVKLVEKSFETDTNLNFQNLSVIGFRILLLKVAGFNLLMTLRLWSS

SEQ ID NO: 118 - DNA, 423 bp, synthetic construct
  source 1..423: mol_type = other DNA
aatatccagaaccctgaccctgccgtgtaccagctgagagactctaaatccagtgacaagtctgtctgcctattcaccgattttgattctcaaacaaatgtgtcacaaagtaaggattctgatgtgtatatcacagacaaaactgtgctagacatgaggtctatggacttcaagagcaacagtgctgtggcctggagcaacaaatctgactttgcatgtgcaaacgccttcaacaacagcattattccagaagacaccttcttccccagcccagaaagttcctgtgatgtcaagctggtcgagaaaagctttgaaacagatacgaacctaaactttcaaaacctgtcagtgattgggttccgaatcctcctcctgaaagtggccgggtttaatctgctcatgacgctgcggctgtggtccagc

SEQ ID NO: 119 - protein, 141 aa, synthetic construct
HIQNPDPAVYQLRDSKSSDKSVCLFTDFDSQTNVSQSKDSDVYITDKTVLDMRSMDFKSNSAVAWSNKSDFACANAFNNSIIPEDTFFPSPESSCDVKLVEKSFETDTNLNFQNLSVIGFRILLLKVAGFNLLMTLRLWSS

SEQ ID NO: 120 - DNA, 423 bp, synthetic construct
  source 1..423: mol_type = other DNA
catatccagaaccctgaccctgccgtgtaccagctgagagactctaaatccagtgacaagtctgtctgcctattcaccgattttgattctcaaacaaatgtgtcacaaagtaaggattctgatgtgtatatcacagacaaaactgtgctagacatgaggtctatggacttcaagagcaacagtgctgtggcctggagcaacaaatctgactttgcatgtgcaaacgccttcaacaacagcattattccagaagacaccttcttccccagcccagaaagttcctgtgatgtcaagctggtcgagaaaagctttgaaacagatacgaacctaaactttcaaaacctgtcagtgattgggttccgaatcctcctcctgaaagtggccgggtttaatctgctcatgacgctgcggctgtggtccagc

SEQ ID NO: 121 - protein, 141 aa, synthetic construct
DIQNPDPAVYQLRDSKSSDKSVCLFTDFDSQTNVSQSKDSDVYITDKTVLDMRSMDFKSNSAVAWSNKSDFACANAFNNSIIPEDTFFPSPESSCDVKLVEKSFETDTNLNFQNLSVIGFRILLLKVAGFNLLMTLRLWSS

SEQ ID NO: 122 - DNA, 423 bp, synthetic construct
  source 1..423: mol_type = other DNA
gatatccagaaccctgaccctgccgtgtaccagctgagagactctaaatccagtgacaagtctgtctgcctattcaccgattttgattctcaaacaaatgtgtcacaaagtaaggattctgatgtgtatatcacagacaaaactgtgctagacatgaggtctatggacttcaagagcaacagtgctgtggcctggagcaacaaatctgactttgcatgtgcaaacgccttcaacaacagcattattccagaagacaccttcttccccagcccagaaagttcctgtgatgtcaagctggtcgagaaaagctttgaaacagatacgaacctaaactttcaaaacctgtcagtgattgggttccgaatcctcctcctgaaagtggccgggtttaatctgctcatgacgctgcggctgtggtccagc

SEQ ID NO: 123 - protein, 141 aa, synthetic construct; identical to SEQ ID NO: 117

SEQ ID NO: 124 - DNA, 423 bp, synthetic construct; identical to SEQ ID NO: 118
  source 1..423: mol_type = other DNA

SEQ ID NO: 125 - protein, 141 aa, synthetic construct; identical to SEQ ID NO: 117

SEQ ID NO: 126 - DNA, 423 bp, synthetic construct; identical to SEQ ID NO: 118
  source 1..423: mol_type = other DNA

SEQ ID NO: 127 - protein, 141 aa, synthetic construct; identical to SEQ ID NO: 117

SEQ ID NO: 128 - DNA, 423 bp, synthetic construct; identical to SEQ ID NO: 118
  source 1..423: mol_type = other DNA

SEQ ID NO: 129 - protein, 141 aa, synthetic construct; identical to SEQ ID NO: 113

SEQ ID NO: 130 - DNA, 423 bp, synthetic construct; identical to SEQ ID NO: 114
  source 1..423: mol_type = other DNA

SEQ ID NO: 131 - protein, 141 aa, synthetic construct; identical to SEQ ID NO: 113

SEQ ID NO: 132 - DNA, 423 bp, synthetic construct; identical to SEQ ID NO: 114
  source 1..423: mol_type = other DNA

SEQ ID NO: 133 - protein, 141 aa, synthetic construct; identical to SEQ ID NO: 121

SEQ ID NO: 134 - DNA, 423 bp, synthetic construct; identical to SEQ ID NO: 122
  source 1..423: mol_type = other DNA

SEQ ID NO: 135 - protein, 141 aa, synthetic construct; identical to SEQ ID NO: 117

SEQ ID NO: 136 - DNA, 423 bp, synthetic construct; identical to SEQ ID NO: 118
  source 1..423: mol_type = other DNA

SEQ ID NO: 137 - protein, 141 aa, synthetic construct; identical to SEQ ID NO: 113

SEQ ID NO: 138 - DNA, 423 bp, synthetic construct; identical to SEQ ID NO: 114
  source 1..423: mol_type = other DNA

SEQ ID NO: 139 - protein, 141 aa, synthetic construct; identical to SEQ ID NO: 113

SEQ ID NO: 140 - DNA, 423 bp, synthetic construct; identical to SEQ ID NO: 114
  source 1..423: mol_type = other DNA

SEQ ID NO: 141 - protein, 141 aa, synthetic construct; identical to SEQ ID NO: 117

SEQ ID NO: 142 - DNA, 423 bp, synthetic construct; identical to SEQ ID NO: 118
  source 1..423: mol_type = other DNA

SEQ ID NO: 143 - protein, 141 aa, synthetic construct; identical to SEQ ID NO: 117

SEQ ID NO: 144 - DNA, 423 bp, synthetic construct; identical to SEQ ID NO: 118
  source 1..423: mol_type = other DNA

SEQ ID NO: 145 - protein, 255 aa, synthetic construct
AQKVTQAQTEISVVEKEDVTLDCVYETRDTTYYLFWYKQPPSGELVFLIRRNSFDEQNEISGRYSWNFQKSTSSFNFTITASQVVDSAVYFCARDQTGANNLFFGTGTRLTVIPYIQNPDPAVYQLRDSKSSDKSVCLFTDFDSQTNVSQSKDSDVYITDKTVLDMRSMDFKSNSAVAWSNKSDFACANAFNNSIIPEDTFFPSPESSCDVKLVEKSFETDTNLNFQNLSVIGFRILLLKVAGFNLLMTLRLWSS

SEQ ID NO: 146 - DNA, 765 bp, synthetic construct
  source 1..765: mol_type = other DNA
gctcagaaggtaactcaagcgcagactgaaatttctgtggtggagaaggaggatgtgaccttggactgtgtgtatgaaacccgtgatactacttattacttattctggtacaagcaaccaccaagtggagaattggttttccttattcgtcggaactcttttgatgagcaaaatgaaataagtggtcggtattcttggaacttccagaaatccaccagttccttcaacttcaccatcacagcctcacaagtcgtggactcagcagtatacttctgtgcccgtgatcaaactggggcaaacaacctcttctttgggactggaacgagactcaccgttattccctatatccagaaccctgaccctgccgtgtaccagctgagagactctaaatccagtgacaagtctgtctgcctattcaccgattttgattctcaaacaaatgtgtcacaaagtaaggattctgatgtgtatatcacagacaaaactgtgctagacatgaggtctatggacttcaagagcaacagtgctgtggcctggagcaacaaatctgactttgcatgtgcaaacgccttcaacaacagcattattccagaagacaccttcttccccagcccagaaagttcctgtgatgtcaagctggtcgagaaaagctttgaaacagatacgaacctaaactttcaaaacctgtcagtgattgggttccgaatcctcctcctgaaagtggccgggtttaatctgctcatgacgctgcggctgtggtccagc

SEQ ID NO: 147 - protein, 260 aa, synthetic construct
AQKVTQAQTEISVVEKEDVTLDCVYETRDTTYYLFWYKQPPSGELVFLIRRNSFDEQNEISGRYSWNFQKSTSSFNFTITASQVVDSAVYFCALSDPRYSGGGADGLTFGKGTHLIIQPYIQNPDPAVYQLRDSKSSDKSVCLFTDFDSQTNVSQSKDSDVYITDKTVLDMRSMDFKSNSAVAWSNKSDFACANAFNNSIIPEDTFFPSPESSCDVKLVEKSFETDTNLNFQNLSVIGFRILLLKVAGFNLLMTLRLWSS

SEQ ID NO: 148 - DNA, 780 bp, synthetic construct
  source 1..780: mol_type = other DNA
gctcagaaggtaactcaagcgcagactgaaatttctgtggtggagaaggaggatgtgaccttggactgtgtgtatgaaacccgtgatactacttattacttattctggtacaagcaaccaccaagtggagaattggttttccttattcgtcggaactcttttgatgagcaaaatgaaataagtggtcggtattcttggaacttccagaaatccaccagttccttcaacttcaccatcacagcctcacaagtcgtggactcagcagtatacttctgtgctctgagtgacccccgttattcaggaggaggtgctgacggactcacctttggcaaagggactcatctaatcatccagccctatatccagaaccctgaccctgccgtgtaccagctgagagactctaaatccagtgacaagtctgtctgcctattcaccgattttgattctcaaacaaatgtgtcacaaagtaaggattctgatgtgtatatcacagacaaaactgtgctagacatgaggtctatggacttcaagagcaacagtgctgtggcctggagcaacaaatctgactttgcatgtgcaaacgccttcaacaacagcattattccagaagacaccttcttccccagcccagaaagttcctgtgatgtcaagctggtcgagaaaagctttgaaacagatacgaacctaaactttcaaaacctgtcagtgattgggttccgaatcctcctcctgaaagtggccgggtttaatctgctcatgacgctgcggctgtggtccagc

SEQ ID NO: 149 - protein, 252 aa, synthetic construct
DQQVKQNSPSLSVQEGRISILNCDYTNSMFDYFLWYKKYPAEGPTFLISISSIKDKNEDGRFTVFLNKSAKHLSLHIVPSQPGDSAVYFCAGYQGGYKLSFGAGTTVTVRANIQNPDPAVYQLRDSKSSDKSVCLFTDFDSQTNVSQSKDSDVYITDKTVLDMRSMDFKSNSAVAWSNKSDFACANAFNNSIIPEDTFFPSPESSCDVKLVEKSFETDTNLNFQNLSVIGFRILLLKVAGFNLLMTLRLWSS

SEQ ID NO: 150 - DNA, 756 bp, synthetic construct
  source 1..756: mol_type = other DNA
gaccagcaagttaagcaaaattcaccatccctgagcgtccaggaaggaagaatttctattctgaactgtgactatactaacagcatgtttgattatttcctatggtacaaaaaataccctgctgaaggtcctacattcctgatatctataagttccattaaggataaaaatgaagatggaagattcactgtcttcttaaacaaaagtgccaagcacctctctctgcacattgtgccctcccagcctggagactctgcagtgtacttctgtgcagggtatcaagggggctacaagctcagctttggagccggaaccacagtaactgtaagagcaaatatccagaaccctgaccctgccgtgtaccagctgagagactctaaatccagtgacaagtctgtctgcctattcaccgattttgattctcaaacaaatgtgtcacaaagtaaggattctgatgtgtatatcacagacaaaactgtgctagacatgaggtctatggacttcaagagcaacagtgctgtggcctggagcaacaaatctgactttgcatgtgcaaacgccttcaacaacagcattattccagaagacaccttcttccccagcccagaaagttcctgtgatgtcaagctggtcgagaaaagctttgaaacagatacgaacctaaactttcaaaacctgtcagtgattgggttccgaatcctcctcctgaaagtggccgggtttaatctgctcatgacgctgcggctgtggtccagc

SEQ ID NO: 151 - protein, 251 aa, synthetic construct
QKEVEQNSGPLSVPEGAIASLNCTYSDRGSQSFFWYRQYSGKSPELIMFIYSNGDKEDGRFTAQLNKASQYVSLLIRDSQPSDSATYLCAVNMPGNMLTFGGGTRLMVKPHIQNPDPAVYQLRDSKSSDKSVCLFTDFDSQTNVSQSKDSDVYITDKTVLDMRSMDFKSNSAVAWSNKSDFACANAFNNSIIPEDTFFPSPESSCDVKLVEKSFETDTNLNFQNLSVIGFRILLLKVAGFNLLMTLRLWSS

SEQ ID NO: 152 - DNA, 753 bp, synthetic construct
  source 1..753: mol_type = other DNA
cagaaggaggtggagcagaattctggacccctcagtgttccagagggagccattgcctctctcaactgcacttacagtgaccgaggttcccagtccttcttctggtacagacaatattctgggaaaagccctgagttgataatgttcatatactccaatggtgacaaagaagatggaaggtttacagcacagctcaataaagccagccagtatgtttctctgctcatcagagactcccagcccagtgattcagccacctacctctgtgccgtgaacatgccaggcaacatgctcacctttggagggggaacaaggttaatggtcaaaccccatatccagaaccctgaccctgccgtgtaccagctgagagactctaaatccagtgacaagtctgtctgcctattcaccgattttgattctcaaacaaatgtgtcacaaagtaaggattctgatgtgtatatcacagacaaaactgtgctagacatgaggtctatggacttcaagagcaacagtgctgtggcctggagcaacaaatctgactttgcatgtgcaaacgccttcaacaacagcattattccagaagacaccttcttccccagcccagaaagttcctgtgatgtcaagctggtcgagaaaagctttgaaacagatacgaacctaaactttcaaaacctgtcagtgattgggttccgaatcctcctcctgaaagtggccgggtttaatctgctcatgacgctgcggctgtggtccagc

SEQ ID NO: 153 - protein, 253 aa, synthetic construct
GEDVEQSLFLSVREGDSSVINCTYTDSSSTYLYWYKQEPGAGLQLLTYIFSNMDMKQDQRLTVLLNKKDKHLSLRIADTQTGDSAIYFCAERGTDSWGKLQFGAGTQVVVTPDIQNPDPAVYQLRDSKSSDKSVCLFTDFDSQTNVSQSKDSDVYITDKTVLDMRSMDFKSNSAVAWSNKSDFACANAFNNSIIPEDTFFPSPESSCDVKLVEKSFETDTNLNFQNLSVIGFRILLLKVAGFNLLMTLRLWSS

SEQ ID NO: 154 - DNA, 759 bp, synthetic construct
  source 1..759: mol_type = other DNA
ggagaggatgtggagcagagtcttttcctgagtgtccgagagggagacagctccgttataaactgcacttacacagacagctcctccacctacttatactggtataagcaagaacctggagcaggtctccagttgctgacgtatattttttcaaatatggacatgaaacaagaccaaagactcactgttctattgaataaaaaggataaacatctgtctctgcgcattgcagacacccagactggggactcagctatctacttctgtgcagagagagggactgacagctgggggaaattgcagtttggagcagggacccaggttgtggtcaccccagatatccagaaccctgaccctgccgtgtaccagctgagagactctaaatccagtgacaagtctgtctgcctattcaccgattttgattctcaaacaaatgtgtcacaaagtaaggattctgatgtgtatatcacagacaaaactgtgctagacatgaggtctatggacttcaagagcaacagtgctgtggcctggagcaacaaatctgactttgcatgtgcaaacgccttcaacaacagcattattccagaagacaccttcttccccagcccagaaagttcctgtgatgtcaagctggtcgagaaaagctttgaaacagatacgaacctaaactttcaaaacctgtcagtgattgggttccgaatcctcctcctgaaagtggccgggtttaatctgctcatgacgctgcggctgtggtccagc

SEQ ID NO: 155 - protein, 254 aa, synthetic construct
SQQGEEDPQALSIQEGENATMNCSYKTSINNLQWYRQNSGRGLVHLILIRSNEREKHSGRLRVTLDTSKKSSSLLITASRAADTASYFCATDDYGGATNKLIFGTGTLLAVQPNIQNPDPAVYQLRDSKSSDKSVCLFTDFDSQTNVSQSKDSDVYITDKTVLDMRSMDFKSNSAVAWSNKSDFACANAFNNSIIPEDTFFPSPESSCDVKLVEKSFETDTNLNFQNLSVIGFRILLLKVAGFNLLMTLRLWSS

SEQ ID NO: 156 - DNA, 762 bp, synthetic construct
  source 1..762: mol_type = other DNA
agtcaacagggagaagaggatcctcaggccttgagcatccaggagggtgaaaatgccaccatgaactgcagttacaaaactagtataaacaatttacagtggtatagacaaaattcaggtagaggccttgtccacctaattttaatacgttcaaatgaaagagagaaacacagtggaagattaagagtcacgcttgacacttccaagaaaagcagttccttgttgatcacggcttcccgggcagcagacactgcttcttacttctgtgctacggacgattatggtggtgctacaaacaagctcatctttggaactggcactctgcttgctgtccagccaaatatccagaaccctgaccctgccgtgtaccagctgagagactctaaatccagtgacaagtctgtctgcctattcaccgattttgattctcaaacaaatgtgtcacaaagtaaggattctgatgtgtatatcacagacaaaactgtgctagacatgaggtctatggacttcaagagcaacagtgctgtggcctggagcaacaaatctgactttgcatgtgcaaacgccttcaacaacagcattattccagaagacaccttcttccccagcccagaaagttcctgtgatgtcaagctggtcgagaaaagctttgaaacagatacgaacctaaactttcaaaacctgtcagtgattgggttccgaatcctcctcctgaaagtggccgggtttaatctgctcatgacgctgcggctgtggtccagc

SEQ ID NO: 157 - protein, 252 aa, synthetic construct
ELKVEQNPLFLSMQEGKNYTIYCNYSTTSDRLYWYRQDPGKSLESLFVLLSNGAVKQEGRLMASLDTKARLSTLHITAAVHDLSATYFCAVDKAAGNKLTFGGGTRVLVKPNIQNPDPAVYQLRDSKSSDKSVCLFTDFDSQTNVSQSKDSDVYITDKTVLDMRSMDFKSNSAVAWSNKSDFACANAFNNSIIPEDTFFPSPESSCDVKLVEKSFETDTNLNFQNLSVIGFRILLLKVAGFNLLMTLRLWSS

SEQ ID NO: 158 - DNA, 756 bp, synthetic construct
  source 1..756: mol_type = other DNA
gagctgaaagtggaacaaaaccctctgttcctgagcatgcaggagggaaaaaactataccatctactgcaattattcaaccacttcagacagactgtattggtacaggcaggatcctgggaaaagtctggaatctctgtttgtgttgctatcaaatggagcagtgaagcaggagggacgattaatggcctcacttgataccaaagcccgtctcagcaccctccacatcacagctgccgtgcatgacctctctgccacctacttctgtgccgtggacaaagctgcaggcaacaagctaacttttggaggaggaaccagggtgctagttaaaccaaatatccagaaccctgaccctgccgtgtaccagctgagagactctaaatccagtgacaagtctgtctgcctattcaccgattttgattctcaaacaaatgtgtcacaaagtaaggattctgatgtgtatatcacagacaaaactgtgctagacatgaggtctatggacttcaagagcaacagtgctgtggcctggagcaacaaatctgactttgcatgtgcaaacgccttcaacaacagcattattccagaagacaccttcttccccagcccagaaagttcctgtgatgtcaagctggtcgagaaaagctttgaaacagatacgaacctaaactttcaaaacctgtcagtgattgggttccgaatcctcctcctgaaagtggccgggtttaatctgctcatgacgctgcggctgtggtccagc

SEQ ID NO: 159 - protein, 245 aa, synthetic construct
KDQVFQPSTVASSEGAVVEIFCNHSVSNAYNFFWYLHFPGCAPRLLVKGSKPSQQGRYNMTYERFSSSLLILQVREADAAVYYCAGSNDYKLSFGAGTTVTVRANIQNPDPAVYQLRDSKSSDKSVCLFTDFDSQTNVSQSKDSDVYITDKTVLDMRSMDFKSNSAVAWSNKSDFACANAFNNSIIPEDTFFPSPESSCDVKLVEKSFETDTNLNFQNLSVIGFRILLLKVAGFNLLMTLRLWSS

SEQ ID NO: 160 - DNA, 735 bp, synthetic construct
  source 1..735: mol_type = other DNA
aaggaccaagtgtttcagccttccacagtggcatcttcagagggagctgtggtggaaatcttctgtaatcactctgtgtccaatgcttacaacttcttctggtaccttcacttcccgggatgtgcaccaagactccttgttaaaggctcaaagccttctcagcagggacgatacaacatgacctatgaacggttctcttcatcgctgctcatcctccaggtgcgggaggcagatgctgctgtttactactgtgctgggtctaacgactacaagctcagctttggagccggaaccacagtaactgtaagagcaaatatccagaaccctgaccctgccgtgtaccagctgagagactctaaatccagtgacaagtctgtctgcctattcaccgattttgattctcaaacaaatgtgtcacaaagtaaggattctgatgtgtatatcacagacaaaactgtgctagacatgaggtctatggacttcaagagcaacagtgctgtggcctggagcaacaaatctgactttgcatgtgcaaacgccttcaacaacagcattattccagaagacaccttcttccccagcccagaaagttcctgtgatgtcaagctggtcgagaaaagctttgaaacagatacgaacctaaactttcaaaacctgtcagtgattgggttccgaatcctcctcctgaaagtggccgggtttaatctgctcatgacgctgcggctgtggtccagc

SEQ ID NO: 161 - protein, 253 aa, synthetic construct
SQQGEEDPQALSIQEGENATMNCSYKTSINNLQWYRQNSGRGLVHLILIRSNEREKHSGRLRVTLDTSKKSSSLLITASRAADTASYFCATDGGGGADGLTFGKGTHLIIQPYIQNPDPAVYQLRDSKSSDKSVCLFTDFDSQTNVSQSKDSDVYITDKTVLDMRSMDFKSNSAVAWSNKSDFACANAFNNSIIPEDTFFPSPESSCDVKLVEKSFETDTNLNFQNLSVIGFRILLLKVAGFNLLMTLRLWSS

SEQ ID NO: 162 - DNA, 759 bp, synthetic construct
  source 1..759: mol_type = other DNA
agtcaacagggagaagaggatcctcaggccttgagcatccaggagggtgaaaatgccaccatgaactgcagttacaaaactagtataaacaatttacagtggtatagacaaaattcaggtagaggccttgtccacctaattttaatacgttcaaatgaaagagagaaacacagtggaagattaagagtcacgcttgacacttccaagaaaagcagttccttgttgatcacggcttcccgggcagcagacactgcttcttacttctgtgctacggacggcggaggaggtgctgacggactcacctttggcaaagggactcatctaatcatccagccctatatccagaaccctgaccctgccgtgtaccagctgagagactctaaatccagtgacaagtctgtctgcctattcaccgattttgattctcaaacaaatgtgtcacaaagtaaggattctgatgtgtatatcacagacaaaactgtgctagacatgaggtctatggacttcaagagcaacagtgctgtggcctggagcaacaaatctgactttgcatgtgcaaacgccttcaacaacagcattattccagaagacaccttcttccccagcccagaaagttcctgtgatgtcaagctggtcgagaaaagctttgaaacagatacgaacctaaactttcaaaacctgtcagtgattgggttccgaatcctcctcctgaaagtggccgggtttaatctgctcatgacgctgcggctgtggtccagc

SEQ ID NO: 163 - protein, 253 aa, synthetic construct
SQQGEEDPQALSIQEGENATMNCSYKTSINNLQWYRQNSGRGLVHLILIRSNEREKHSGRLRVTLDTSKKSSSLLITASRAADTASYFCATDSGGGADGLTFGKGTHLIIQPYIQNPDPAVYQLRDSKSSDKSVCLFTDFDSQTNVSQSKDSDVYITDKTVLDMRSMDFKSNSAVAWSNKSDFACANAFNNSIIPEDTFFPSPESSCDVKLVEKSFETDTNLNFQNLSVIGFRILLLKVAGFNLLMTLRLWSS

SEQ ID NO: 164 - DNA, 759 bp, synthetic construct
  source 1..759: mol_type = other DNA
agtcaacagggagaagaggatcctcaggccttgagcatccaggagggtgaaaatgccaccatgaactgcagttacaaaactagtataaacaatttacagtggtatagacaaaattcaggtagaggccttgtccacctaattttaatacgttcaaatgaaagagagaaacacagtggaagattaagagtcacgcttgacacttccaagaaaagcagttccttgttgatcacggcttcccgggcagcagacactgcttcttacttctgtgctacggattcaggaggaggtgctgacggactcacctttggcaaagggactcatctaatcatccagccctatatccagaaccctgaccctgccgtgtaccagctgagagactctaaatccagtgacaagtctgtctgcctattcaccgattttgattctcaaacaaatgtgtcacaaagtaaggattctgatgtgtatatcacagacaaaactgtgctagacatgaggtctatggacttcaagagcaacagtgctgtggcctggagcaacaaatctgactttgcatgtgcaaacgccttcaacaacagcattattccagaagacaccttcttccccagcccagaaagttcctgtgatgtcaagctggtcgagaaaagctttgaaacagatacgaacctaaactttcaaaacctgtcagtgattgggttccgaatcctcctcctgaaagtggccgggtttaatctgctcatgacgctgcggctgtggtccagc

SEQ ID NO: 165 - protein, 254 aa, synthetic construct
DQQVKQNSPSLSVQEGRISILNCDYTNSMFDYFLWYKKYPAEGPTFLISISSIKDKNEDGRFTVFLNKSAKHLSLHIVPSQPGDSAVYFCAASYAGSARQLTFGSGTQLTVLPDIQNPDPAVYQLRDSKSSDKSVCLFTDFDSQTNVSQSKDSDVYITDKTVLDMRSMDFKSNSAVAWSNKSDFACANAFNNSIIPEDTFFPSPESSCDVKLVEKSFETDTNLNFQNLSVIGFRILLLKVAGFNLLMTLRLWSS

SEQ ID NO: 166 - DNA, 762 bp, synthetic construct
  source 1..762: mol_type = other DNA
gaccagcaagttaagcaaaattcaccatccctgagcgtccaggaaggaagaatttctattctgaactgtgactatactaacagcatgtttgattatttcctatggtacaaaaaataccctgctgaaggtcctacattcctgatatctataagttccattaaggataaaaatgaagatggaagattcactgtcttcttaaacaaaagtgccaagcacctctctctgcacattgtgccctcccagcctggagactctgcagtgtacttctgtgcagcaagctacgccggttctgcaaggcaactgacctttggatctgggacacaattgactgttttacctgatatccagaaccctgaccctgccgtgtaccagctgagagactctaaatccagtgacaagtctgtctgcctattcaccgattttgattctcaaacaaatgtgtcacaaagtaaggattctgatgtgtatatcacagacaaaactgtgctagacatgaggtctatggacttcaagagcaacagtgctgtggcctggagcaacaaatctgactttgcatgtgcaaacgccttcaacaacagcattattccagaagacaccttcttccccagcccagaaagttcctgtgatgtcaagctggtcgagaaaagctttgaaacagatacgaacctaaactttcaaaacctgtcagtgattgggttccgaatcctcctcctgaaagtggccgggtttaatctgctcatgacgctgcggctgtggtccagc

SEQ ID NO: 167 - protein, 252 aa, synthetic construct
QKEVEQNSGPLSVPEGAIASLNCTYSDRGSQSFFWYRQYSGKSPELIMFIYSNGDKEDGRFTAQLNKASQYVSLLIRDSQPSDSATYLCARKKTSYDKVIFGPGTSLSVIPNIQNPDPAVYQLRDSKSSDKSVCLFTDFDSQTNVSQSKDSDVYITDKTVLDMRSMDFKSNSAVAWSNKSDFACANAFNNSIIPEDTFFPSPESSCDVKLVEKSFETDTNLNFQNLSVIGFRILLLKVAGFNLLMTLRLWSS

SEQ ID NO: 168 - DNA, 756 bp, synthetic construct
  source 1..756: mol_type = other DNA
cagaaggaggtggagcagaattctggacccctcagtgttccagagggagccattgcctctctcaactgcacttacagtgaccgaggttcccagtccttcttctggtacagacaatattctgggaaaagccctgagttgataatgttcatatactccaatggtgacaaagaagatggaaggtttacagcacagctcaataaagccagccagtatgtttctctgctcatcagagactcccagcccagtgattcagccacctacctctgtgcccgcaagaaaacctcctacgacaaggtgatatttgggccagggacaagcttatcagtcattccaaatatccagaaccctgaccctgccgtgtaccagctgagagactctaaatccagtgacaagtctgtctgcctattcaccgattttgattctcaaacaaatgtgtcacaaagtaaggattctgatgtgtatatcacagacaaaactgtgctagacatgaggtctatggacttcaagagcaacagtgctgtggcctggagcaacaaatctgactttgcatgtgcaaacgccttcaacaacagcattattccagaagacaccttcttccccagcccagaaagttcctgtgatgtcaagctggtcgagaaaagctttgaaacagatacgaacctaaactttcaaaacctgtcagtgattgggttccgaatcctcctcctgaaagtggccgggtttaatctgctcatgacgctgcggctgtggtccagc

SEQ ID NO: 169 - protein, 254 aa, synthetic construct
GNSVTQMEGPVTLSEEAFLTINCTYTATGYPSLFWYVQYPGEGLQLLLKATKADDKGSNKGFEATYRKETTSFHLEKGSVQVSDSAVYFCALPAGGGADGLTFGKGTHLIIQPYIQNPDPAVYQLRDSKSSDKSVCLFTDFDSQTNVSQSKDSDVYITDKTVLDMRSMDFKSNSAVAWSNKSDFACANAFNNSIIPEDTFFPSPESSCDVKLVEKSFETDTNLNFQNLSVIGFRILLLKVAGFNLLMTLRLWSS

SEQ ID NO: 170 - DNA, 762 bp, synthetic construct
  source 1..762: mol_type = other DNA
ggaaattcagtgacccagatggaagggccagtgactctctcagaagaggccttcctgactataaactgcacgtacacagccacaggatacccttcccttttctggtatgtccaatatcctggagaaggtctacagctcctcctgaaagccacgaaggctgatgacaagggaagcaacaaaggttttgaagccacataccgtaaagaaaccacttctttccacttggagaaaggctcagttcaagtgtcagactcagcggtgtacttctgtgctctgcccgcaggaggaggtgctgacggactcacctttggcaaagggactcatctaatcatccagccctatatccagaaccctgaccctgccgtgtaccagctgagagactctaaatccagtgacaagtctgtctgcctattcaccgattttgattctcaaacaaatgtgtcacaaagtaaggattctgatgtgtatatcacagacaaaactgtgctagacatgaggtctatggacttcaagagcaacagtgctgtggcctggagcaacaaatctgactttgcatgtgcaaacgccttcaacaacagcattattccagaagacaccttcttccccagcccagaaagttcctgtgatgtcaagctggtcgagaaaagctttgaaacagatacgaacctaaactttcaaaacctgtcagtgattgggttccgaatcctcctcctgaaagtggccgggtttaatctgctcatgacgctgcggctgtggtccagc

SEQ ID NO: 171 - protein, 253 aa, synthetic construct
SQQGEEDPQALSIQEGENATMNCSYKTSINNLQWYRQNSGRGLVHLILIRSNEREKHSGRLRVTLDTSKKSSSLLITASRAADTASYFCATDRTGGYNKLIFGAGTRLAVHPYIQNPDPAVYQLRDSKSSDKSVCLFTDFDSQTNVSQSKDSDVYITDKTVLDMRSMDFKSNSAVAWSNKSDFACANAFNNSIIPEDTFFPSPESSCDVKLVEKSFETDTNLNFQNLSVIGFRILLLKVAGFNLLMTLRLWSS

SEQ ID NO: 172 - DNA, 759 bp, synthetic construct
  source 1..759: mol_type = other DNA
agtcaacagggagaagaggatcctcaggccttgagcatccaggagggtgaaaatgccaccatgaactgcagttacaaaactagtataaacaatttacagtggtatagacaaaattcaggtagaggccttgtccacctaattttaatacgttcaaatgaaagagagaaacacagtggaagattaagagtcacgcttgacacttccaagaaaagcagttccttgttgatcacggcttcccgggcagcagacactgcttcttacttctgtgctacggaccgaactggtggctacaataagctgatttttggagcagggaccaggctggctgtacacccatatatccagaaccctgaccctgccgtgtaccagctgagagactctaaatccagtgacaagtctgtctgcctattcaccgattttgattctcaaacaaatgtgtcacaaagtaaggattctgatgtgtatatcacagacaaaactgtgctagacatgaggtctatggacttcaagagcaacagtgctgtggcctggagcaacaaatctgactttgcatgtgcaaacgccttcaacaacagcattattccagaagacaccttcttccccagcccagaaagttcctgtgatgtcaagctggtcgagaaaagctttgaaacagatacgaacctaaactttcaaaacctgtcagtgattgggttccgaatcctcctcctgaaagtggccgggtttaatctgctcatgacgctgcggctgtggtccagc

SEQ ID NO: 173 - protein, 252 aa, synthetic construct
ILNVEQSPQSLHVQEGDSTNFTCSFPSSNFYALHWYRWETAKSPEALFVMTLNGDEKKKGRISATLNTKEGYSYLYIKGSQPEDSATYLCAFNNQGGKLIFGQGTELSVKPNIQNPDPAVYQLRDSKSSDKSVCLFTDFDSQTNVSQSKDSDVYITDKTVLDMRSMDFKSNSAVAWSNKSDFACANAFNNSIIPEDTFFPSPESSCDVKLVEKSFETDTNLNFQNLSVIGFRILLLKVAGFNLLMTLRLWSS

SEQ ID NO: 174 - DNA, 756 bp, synthetic construct
  source 1..756: mol_type = other DNA
atactgaacgtggaacaaagtcctcagtcactgcatgttcaggagggagacagcaccaatttcacctgcagcttcccttccagcaatttttatgccttacactggtacagatgggaaactgcaaaaagccccgaggccttgtttgtaatgactttaaatggggatgaaaagaagaaaggacgaataagtgccactcttaataccaaggagggttacagctatttgtacatcaaaggatcccagcctgaagactcagccacatacctctgtgcctttaataaccagggaggaaagcttatcttcggacagggaacggagttatctgtgaaacccaatatccagaaccctgaccctgccgtgtaccagctgagagactctaaatccagtgacaagtctgtctgcctattcaccgattttgattctcaaacaaatgtgtcacaaagtaaggattctgatgtgtatatcacagacaaaactgtgctagacatgaggtctatggacttcaagagcaacagtgctgtggcctggagcaacaaatctgactttgcatgtgcaaacgccttcaacaacagcattattccagaagacaccttcttccccagcccagaaagttcctgtgatgtcaagctggtcgagaaaagctttgaaacagatacgaacctaaactttcaaaacctgtcagtgattgggttccgaatcctcctcctgaaagtggccgggtttaatctgctcatgacgctgcggctgtggtccagc

SEQ ID NO: 175 - protein, 253 aa, synthetic construct
AQSVTQLDSHVSVSEGTPVLLRCNYSSSYSPSLFWYVQHPNKGLQLLLKYTSAATLVKGINGFEAEFKKSETSFHLTKPSAHMSDAAEYFCVVSVWTDKLIFGTGTRLQVFPNIQNPDPAVYQLRDSKSSDKSVCLFTDFDSQTNVSQSKDSDVYITDKTVLDMRSMDFKSNSAVAWSNKSDFACANAFNNSIIPEDTFFPSPESSCDVKLVEKSFETDTNLNFQNLSVIGFRILLLKVAGFNLLMTLRLWSS

SEQ ID NO: 176 - DNA, 759 bp, synthetic construct
  source 1..759: mol_type = other DNA
gcccagtcggtgacccagcttgacagccacgtctctgtctctgaaggaaccccggtgctgctgaggtgcaactactcatcttcttattcaccatctctcttctggtatgtgcaacaccccaacaaaggactccagcttctcctgaagtacacatcagcggccaccctggttaaaggcatcaacggttttgaggctgaatttaagaagagtgaaacctccttccacctgacgaaaccctcagcccatatgagcgacgcggctgagtacttctgtgttgtgagtgtatggaccgacaagctcatctttgggactgggaccagattacaagtctttccaaatatccagaaccctgaccctgccgtgtaccagctgagagactctaaatccagtgacaagtctgtctgcctattcaccgattttgattctcaaacaaatgtgtcacaaagtaaggattctgatgtgtatatcacagacaaaactgtgctagacatgaggtctatggacttcaagagcaacagtgctgtggcctggagcaacaaatctgactttgcatgtgcaaacgccttcaacaacagcattattccagaagacaccttcttccccagcccagaaagttcctgtgatgtcaagctggtcgagaaaagctttgaaacagatacgaacctaaactttcaaaacctgtcagtgattgggttccgaatcctcctcctgaaagtggccgggtttaatctgctcatgacgctgcggctgtggtccagc

SEQ ID NO: 177 - protein, 5 aa, synthetic construct
MDHEN

SEQ ID NO: 178 - protein, 6 aa, synthetic construct
SYDVKM

SEQ ID NO: 179 - protein, 17 aa, synthetic construct
ASSPPHLASGASTDTQY

SEQ ID NO: 180 - protein, 5 aa, synthetic construct
SGDLS

SEQ ID NO: 181 - protein, 6 aa, synthetic construct
YYNGEE

SEQ ID NO: 182 - protein, 15 aa, synthetic construct
ASSPRGGDSILDTQY

SEQ ID NO: 183 - protein, 5 aa, synthetic construct
MNHEY

SEQ ID NO: 184 - protein, 6 aa, synthetic construct
SMNVEV

SEQ ID NO: 185 - protein, 12 aa, synthetic construct
ASSTRDRDNEQF

SEQ ID NO: 186 - protein, 5 aa, synthetic construct
LGHNT

SEQ ID NO: 187 - protein, 6 aa, synthetic construct
FRNRAP

SEQ ID NO: 188 - protein, 12 aa, synthetic construct
ASGPEGLDNEQF

SEQ ID NO: 189 - protein, 6 aa, synthetic construct
DFQATT

SEQ ID NO: 190 - protein, 7 aa, synthetic construct
SNEGSKA

SEQ ID NO: 191 - protein, 11 aa, synthetic construct
SARFANYYEQY

SEQ ID NO: 192 - protein, 5 aa, synthetic construct
MGHDK

SEQ ID NO: 193 - protein, 6 aa, synthetic construct
SYGVNS

SEQ ID NO: 194 - protein, 13 aa, synthetic construct
ASSDPVHGDYGYT

SEQ ID NO: 195 - protein, 5 aa, synthetic construct
KGHSY

SEQ ID NO: 196 - protein, 6 aa, synthetic construct
FQNENV

SEQ ID NO: 197 - protein, 11 aa, synthetic construct
ASSPHHRYEQY

SEQ ID NO: 198 - protein, 5 aa, synthetic construct
MNHEY

SEQ ID NO: 199 - protein, 6 aa, synthetic construct
SMNVEV

SEQ ID NO: 200 - protein, 11 aa, synthetic construct
ASSTSPYNEQF

SEQ ID NO: 201 - protein, 5 aa, synthetic construct
SGDLS

SEQ ID NO: 202 - protein, 6 aa, synthetic construct
YYNGEE

SEQ ID NO: 203 - protein, 13 aa, synthetic construct
ASSLHRDSDTEAF

SEQ ID NO: 204 - protein, 5 aa, synthetic construct
SGDLS

SEQ ID NO: 205 - protein, 6 aa, synthetic construct
YYNGEE

SEQ ID NO: 206 - protein, 13 aa, synthetic construct
ASSHGRDSTDTQY

SEQ ID NO: 207 - protein, 5 aa, synthetic construct
SGHTA

SEQ ID NO: 208 - protein, 6 aa, synthetic construct
FQGNSA

SEQ ID NO: 209 - protein, 11 aa, synthetic construct
ASSPGGNYGYT

SEQ ID NO: 210 - protein, 5 aa, synthetic construct
SGDLS

SEQ ID NO: 211 - protein, 6 aa, synthetic construct
YYNGEE

SEQ ID NO: 212 - protein, 10 aa, synthetic construct
ASSLGDSEQF

SEQ ID NO: 213 - protein, 5 aa, synthetic construct
SGHTA

SEQ ID NO: 214 - protein, 6 aa, synthetic construct
FQGNSA

SEQ ID NO: 215 - protein, 14 aa, synthetic construct
ASSFGTSGDQYEQY

SEQ ID NO: 216 - protein, 5 aa, synthetic construct
SGHNT

SEQ ID NO: 217 - protein, 6 aa, synthetic construct
YYREEE

SEQ ID NO: 218 - protein, 11 aa, synthetic construct
ASSLQTGDEQY

SEQ ID NO: 219 - protein, 5 aa, synthetic construct
MNHEY

SEQ ID NO: 220 - protein, 6 aa, synthetic construct
SMNVEV

SEQ ID NO: 221 - protein, 13 aa, synthetic construct
ASSSGTGGGAEAF

SEQ ID NO: 222 - protein, 6 aa, synthetic construct
DFQATT

SEQ ID NO: 223 - protein, 7 aa, synthetic construct
SNEGSKA

SEQ ID NO: 224 - protein, 12 aa, synthetic construct
SANRDFGIYEQY

SEQ ID NO: 225 - protein, 93 aa, synthetic construct
DVKVTQSSRYLVKRTGEKVFLECVQDMDHENMFWYRQDPGLGLRLIYFSYDVKMKEKGDIPEGYSVSREKKERFSLILESASTNQTSMYLCAS

SEQ ID NO: 226 - DNA, 279 bp, synthetic construct
  source 1..279: mol_type = other DNA
gatgtgaaagtaacccagagctcgagatatctagtcaaaaggacgggagagaaagtttttctggaatgtgtccaggatatggaccatgaaaatatgttctggtatcgacaagacccaggtctggggctacggctgatctatttctcatatgatgttaaaatgaaagaaaaaggagatattcctgaggggtacagtgtctctagagagaagaaggagcgcttctccctgattctggagtccgccagcaccaaccagacatctatgtacctctgtgccagc

SEQ ID NO: 227-228 - skipped (2 entries)

SEQ ID NO: 229 - protein, 16 aa, synthetic construct
STDTQYFGPGTRLTVL

SEQ ID NO: 230 - DNA, 48 bp, synthetic construct
  source 1..48: mol_type = other DNA
agcacagatacgcagtattttggcccaggcacccggctgacagtgctc

SEQ ID NO: 231 - protein, 94 aa, synthetic construct
DSGVTQTPKHLITATGQRVTLRCSPRSGDLSVYWYQQSLDQGLQFLIQYYNGEERAKGNILERFSAQQFPDLHSELNLSSLELGDSALYFCASS

SEQ ID NO: 232 - DNA, 282 bp, synthetic construct
  source 1..282: mol_type = other DNA
gattctggagtcacacaaaccccaaagcacctgatcacagcaactggacagcgagtgacgctgagatgctcccctaggtctggagacctctctgtgtactggtaccaacagagcctggaccagggcctccagttcctcattcagtattataatggagaagagagagcaaaaggaaacattcttgaacgattctccgcacaacagttccctgacttgcactctgaactaaacctgagctctctggagctgggggactcagctttgtatttctgtgccagcagc

SEQ ID NO: 233-234 - skipped (2 entries)

SEQ ID NO: 235 - protein, 14 aa, synthetic construct
DTQYFGPGTRLTVL

SEQ ID NO: 236 - DNA, 42 bp, synthetic construct
  source 1..42: mol_type = other DNA
gatacgcagtattttggcccaggcacccggctgacagtgctc

SEQ ID NO: 237 - protein, 93 aa, synthetic construct
EAQVTQNPRYLITVTGKKLTVTCSQNMNHEYMSWYRQDPGLGLRQIYYSMNVEVTDKGDVPEGYKVSRKEKRNFPLILESPSPNQTSLYFCAS

SEQ ID NO: 238 - DNA, 279 bp, synthetic construct
  source 1..279: mol_type = other DNA
gaagcccaagtgacccagaacccaagatacctcatcacagtgactggaaagaagttaacagtgacttgttctcagaatatgaaccatgagtatatgtcctggtatcgacaagacccagggctgggcttaaggcagatctactattcaatgaatgttgaggtgactgataagggagatgttcctgaagggtacaaagtctctcgaaaagagaagaggaatttccccctgatcctggagtcgcccagccccaaccagacctctctgtacttctgtgccagc

SEQ ID NO: 239-240 - skipped (2 entries)

SEQ ID NO: 241 - protein, 14 aa, synthetic construct
NEQFFGPGTRLTVL

SEQ ID NO: 242 - DNA, 42 bp, synthetic construct
  source 1..42: mol_type = other DNA
aatgagcagttcttcgggccagggacacggctcaccgtgcta

SEQ ID NO: 243 - protein, 95 aa, synthetic construct
DARVTQTPRDKVTEMGQEVTMRCQPILGHNTVFWYRQTMMQGLELLAYFRNRAPLDDSGMPKDRFSAEMPDATLATLKIQPSEPRDSAVYFCASG

SEQ ID NO: 244 - DNA, 285 bp, synthetic construct
  source 1..285: mol_type = other DNA
gatgctagagtcacccagacaccaagggacaaggtgacagagatgggacaagaagtaacaatgagatgtcagccaattttaggccacaatactgttttctggtacagacagaccatgatgcaaggactggagttgctggcttacttccgcaaccgggctcctctagatgattcggggatgccgaaggatcgattctcagcagagatgcctgatgcaactttagccactctgaagatccagccctcagaacccagggactcagctgtgtatttttgtgctagtggt

SEQ ID NO: 245-246 - skipped (2 entries)

SEQ ID NO: 247 - protein, 14 aa, synthetic construct
NEQFFGPGTRLTVL

SEQ ID NO: 248 - DNA, 42 bp, synthetic construct; identical to SEQ ID NO: 242
  source 1..42: mol_type = other DNA

SEQ ID NO: 249 - protein, 96 aa, synthetic construct
GAVVSQHPSWVICKSGTSVKIECRSLDFQATTMFWYRQFPKQSLMLMATSNEGSKATYEQGVEKDKFLINHASLTLSTLTVTSAHPEDSSFYICSA

SEQ ID NO: 250 - DNA, 288 bp, synthetic construct
  source 1..288: mol_type = other DNA
ggtgctgtcgtctctcaacatccgagctgggttatctgtaagagtggaacctctgtgaagatcgagtgccgttccctggactttcaggccacaactatgttttggtatcgtcagttcccgaaacagagtctcatgctgatggcaacttccaatgagggctccaaggccacatacgagcaaggcgtcgagaaggacaagtttctcatcaaccatgcaagcctgaccttgtccactctgacagtgaccagtgcccatcctgaagacagcagcttctacatctgcagtgct

SEQ ID NO: 251 - protein, 14 aa, synthetic construct
YEQYFGPGTRLTVT

SEQ ID NO: 252 - DNA, 42 bp, synthetic construct
  source 1..42: mol_type = other DNA
tacgagcagtacttcgggccgggcaccaggctcacggtcaca

SEQ ID NO: 253 - protein, 94 aa, synthetic construct
EADIYQTPRYLVIGTGKKITLECSQTMGHDKMYWYQQDPGMELHLIHYSYGVNSTEKGDLSSESTVSRIRTEHFPLTLESARPSHTSQYLCASS

SEQ ID NO: 254 - DNA, 282 bp, synthetic construct
  source 1..282: mol_type = other DNA
gaagctgacatctaccagaccccaagataccttgttatagggacaggaaagaagatcactctggaatgttctcaaaccatgggccatgacaaaatgtactggtatcaacaagatccaggaatggaactacacctcatccactattcctatggagttaattccacagagaagggagatctttcctctgagtcaacagtctccagaataaggacggagcattttcccctgaccctggagtctgccaggccctcacatacctctcagtacctctgtgccagcagt

SEQ ID NO: 255 - protein, 14 aa, synthetic construct
YGYTFGSGTRLTVV

SEQ ID NO: 256 - DNA, 42 bp, synthetic construct
  source 1..42: mol_type = other DNA
tatggctacaccttcggttcggggaccaggttaaccgttgta

SEQ ID NO: 257 - protein, 95 aa, synthetic construct
GEEVAQTPKHLVRGEGQKAKLYCAPIKGHSYVFWYQQVLKNEFKFLISFQNENVFDETGMPKERFSAKCLPNSPCSLEIQATKLEDSAVYFCASS

SEQ ID NO: 258 - DNA, 285 bp, synthetic construct
  source 1..285: mol_type = other DNA
ggtgaagaagtcgcccagactccaaaacatcttgtcagaggggaaggacagaaagcaaaattatattgtgccccaataaaaggacacagttatgttttttggtaccaacaggtcctgaaaaacgagttcaagttcttgatttccttccagaatgaaaatgtctttgatgaaacaggtatgcccaaggaaagattttcagctaagtgcctcccaaattcaccctgtagccttgagatccaggctacgaagcttgaggattcagcagtgtatttttgtgccagcagc

SEQ ID NO: 259-260 - skipped (2 entries)

SEQ ID NO: 261 - protein, 14 aa, synthetic construct
YEQYFGPGTRLTVT

SEQ ID NO: 262 - DNA, 42 bp, synthetic construct; identical to SEQ ID NO: 252
  source 1..42: mol_type = other DNA

SEQ ID NO: 263 - protein, 93 aa, synthetic construct; identical to SEQ ID NO: 237

SEQ ID NO: 264 - DNA, 279 bp, synthetic construct; identical to SEQ ID NO: 238
  source 1..279: mol_type = other DNA

SEQ ID NO: 265-266 - skipped (2 entries)

SEQ ID NO: 267 - protein, 15 aa, synthetic construct
YNEQFFGPGTRLTVL

SEQ ID NO: 268 - DNA, 45 bp, synthetic construct
  source 1..45: mol_type = other DNA
tacaatgagcagttcttcgggccagggacacggctcaccgtgcta

SEQ ID NO: 269 - protein, 94 aa, synthetic construct; identical to SEQ ID NO: 231

SEQ ID NO: 270 - DNA, 282 bp, synthetic construct; identical to SEQ ID NO: 232
  source 1..282: mol_type = other DNA

SEQ ID NO: 271-272 - skipped (2 entries)

SEQ ID NO: 273 - protein, 14 aa, synthetic construct
TEAFFGQGTRLTVV

SEQ ID NO: 274 - DNA, 42 bp, synthetic construct
  source 1..42: mol_type = other DNA
actgaagctttctttggacaaggcaccagactcacagttgta

SEQ ID NO: 275 - protein, 94 aa, synthetic construct; identical to SEQ ID NO: 231

SEQ ID NO: 276 - DNA, 282 bp, synthetic construct; identical to SEQ ID NO: 232
  source 1..282: mol_type = other DNA

SEQ ID NO: 277-278 - skipped (2 entries)

SEQ ID NO: 279 - protein, 16 aa, synthetic construct
STDTQYFGPGTRLTVL

SEQ ID NO: 280 - DNA, 48 bp, synthetic construct; identical to SEQ ID NO: 230
  source 1..48: mol_type = other DNA

SEQ ID NO: 281 - protein, 94 aa, synthetic construct
GAGVSQSPSNKVTEKGKDVELRCDPISGHTALYWYRQRLGQGLEFLIYFQGNSAPDKSGLPSDRFSAERTGESVSTLTIQRTQQEDSAVYLCAS

SEQ ID NO: 282 - DNA, 282 bp, synthetic construct
  source 1..282: mol_type = other DNA
ggagctggagtctcccagtcccccagtaacaaggtcacagagaagggaaaggatgtagagctcaggtgtgatccaatttcaggtcatactgccctttactggtaccgacagaggctggggcagggcctggagtttttaatttacttccaaggcaacagtgcaccagacaaatcagggctgcccagtgatcgcttctctgcagagaggactggggaatccgtctccactctgacgatccagcgcacacagcaggaggactcggccgtgtatctctgtgccagc

SEQ ID NO: 283-284 - skipped (2 entries)

SEQ ID NO: 285 - protein, 15 aa, synthetic construct
NYGYTFGSGTRLTVV

SEQ ID NO: 286 - DNA, 45 bp, synthetic construct
  source 1..45: mol_type = other DNA
aactatggctacaccttcggttcggggaccaggttaaccgttgta

SEQ ID NO: 287 - protein, 94 aa, synthetic construct; identical to SEQ ID NO: 231

SEQ ID NO: 288 - DNA, 282 bp, synthetic construct; identical to SEQ ID NO: 232
  source 1..282: mol_type = other DNA

SEQ ID NO: 289-290 - skipped (2 entries)

SEQ ID NO: 291 - protein, 13 aa, synthetic construct
EQFFGPGTRLTVL

SEQ ID NO: 292 - DNA, 39 bp, synthetic construct
  source 1..39: mol_type = other DNA
gagcagttcttcgggccagggacacggctcaccgtgcta

SEQ ID NO: 293 - protein, 95 aa, synthetic construct
GAGVSQSPSNKVTEKGKDVELRCDPISGHTALYWYRQSLGQGLEFLIYFQGNSAPDKSGLPSDRFSAERTGGSVSTLTIQRTQQEDSAVYLCASS

SEQ ID NO: 294 - DNA, 285 bp, synthetic construct
  source 1..285: mol_type = other DNA
ggagctggagtctcccagtcccccagtaacaaggtcacagagaagggaaaggatgtagagctcaggtgtgatccaatttcaggtcatactgccctttactggtaccgacagagcctggggcagggcctggagtttttaatttacttccaaggcaacagtgcaccagacaaatcagggctgcccagtgatcgcttctctgcagagaggactgggggatccgtctccactctgacgatccagcgcacacagcaggaggactcggccgtgtatctctgtgccagcagc

SEQ ID NO: 295 - protein, 4 aa, synthetic construct
GTSG

SEQ ID NO: 296 - DNA, 12 bp, synthetic construct
  source 1..12: mol_type = other DNA
gggactagcggg

SEQ ID NO: 297 - protein, 14 aa, synthetic construct
YEQYFGPGTRLTVT

SEQ ID NO: 298 - DNA, 42 bp, synthetic construct; identical to SEQ ID NO: 252
  source 1..42: mol_type = other DNA

SEQ ID NO: 299 - protein, 94 aa, synthetic construct
ETGVTQSPTHLIKTRGQQVTLRCSSQSGHNTVSWYQQALGQGPQFIFQYYREEENGRGNFPPRFSGLQFPNYSSELNVNALELDDSALYLCASS

SEQ ID NO: 300 - DNA, 282 bp, synthetic construct
  source 1..282: mol_type = other DNA
gagactggagtcacccaaagtcccacacacctgatcaaaacgagaggacagcaagtgactctgagatgctcttctcagtctgggcacaacactgtgtcctggtaccaacaggccctgggtcaggggccccagtttatctttcagtattatagggaggaagagaatggcagaggaaacttccctcctagattctcaggtctccagttccctaattatagctctgagctgaatgtgaacgccttggagctggacgactcggccctgtatctctgtgccagcagc

SEQ ID NO: 301-302 - skipped (2 entries)

SEQ ID NO: 303 - protein, 13 aa, synthetic construct
EQYFGPGTRLTVT

SEQ ID NO: 304 - DNA, 39 bp, synthetic construct
  source 1..39: mol_type = other DNA
gagcagtacttcgggccgggcaccaggctcacggtcaca

SEQ ID NO: 305 - protein, 94 aa, synthetic construct
EAQVTQNPRYLITVTGKKLTVTCSQNMNHEYMSWYRQDPGLGLRQIYYSMNVEVTDKGDVPEGYKVSRKEKRNFPLILESPSPNQTSLYFCASS

SEQ ID NO: 306 - DNA, 282 bp, synthetic construct
  source 1..282: mol_type = other DNA
gaagcccaagtgacccagaacccaagatacctcatcacagtgactggaaagaagttaacagtgacttgttctcagaatatgaaccatgagtatatgtcctggtatcgacaagacccagggctgggcttaaggcagatctactattcaatgaatgttgaggtgactgataagggagatgttcctgaagggtacaaagtctctcgaaaagagaagaggaatttccccctgatcctggagtcgcccagccccaaccagacctctctgtacttctgtgccagcagt

SEQ ID NO: 307-308 - skipped (2 entries)

SEQ ID NO: 309 - protein, 13 aa, synthetic construct
EAFFGQGTRLTVV

SEQ ID NO: 310 - DNA, 39 bp, synthetic construct
  source 1..39: mol_type = other DNA
gaagctttctttggacaaggcaccagactcacagttgta

SEQ ID NO: 311 - protein, 95 aa, synthetic construct
GAVVSQHPSWVICKSGTSVKIECRSLDFQATTMFWYRQFPKQSLMLMATSNEGSKATYEQGVEKDKFLINHASLTLSTLTVTSAHPEDSSFYICS

SEQ ID NO: 312 - DNA, 285 bp, synthetic construct
  source 1..285: mol_type = other DNA
ggtgctgtcgtctctcaacatccgagctgggttatctgtaagagtggaacctctgtgaagatcgagtgccgttccctggactttcaggccacaactatgttttggtatcgtcagttcccgaaacagagtctcatgctgatggcaacttccaatgagggctccaaggccacatacgagcaaggcgtcgagaaggacaagtttctcatcaaccatgcaagcctgaccttgtccactctgacagtgaccagtgcccatcctgaagacagcagcttctacatctgcagt

SEQ ID NO: 313-314 - skipped (2 entries)

SEQ ID NO: 315 - protein, 14 aa, synthetic construct
YEQYFGPGTRLTVT

SEQ ID NO: 316 - DNA, 42 bp, synthetic construct; identical to SEQ ID NO: 252
  source 1..42: mol_type = other DNA

SEQ ID NO: 317 - protein, 179 aa, synthetic construct
EDLKNVFPPEVAVFEPSEAEISHTQKATLVCLATGFYPDHVELSWWVNGKEVHSGVSTDPQPLKEQPALNDSRYCLSSRLRVSATFWQNPRNHFRCQVQFYGLSENDEWTQDRAKPVTQIVSAEAWGRADCGFTSESYQQGVLSATILYEILLGKATLYAVLVSALVLMAMVKRKDSRG

SEQ ID NO: 318 - DNA, 536 bp, synthetic construct
  source 1..536: mol_type = other DNA
aggacctgaaaaacgtgttcccacccgaggtcgctgtgtttgagccatcagaagcagagatctcccacacccaaaaggccacactggtgtgcctggccacaggcttctaccccgaccacgtggagctgagctggtgggtgaatgggaaggaggtgcacagtggggtcagcacagacccgcagcccctcaaggagcagcccgccctcaatgactccagatactgcctgtcctcccgcctgagggtctcggccaccttctggcagaacccccgcaaccacttccgctgtcaagtccagttctacgggctctcggagaatgacgagtggacccaggatagggccaaacctgtcacccagatcgtcagcgccgaggcctggggtagagcagactgtggcttcacctccgagtcttaccagcaaggggtcctgtctgccaccatcctctatgagatcttgctagggaaggccaccttgtatgccgtgctggtcagtgccctcgtgctgatggccatggtcaagagaaaggattccagaggc

SEQ ID NO: 319 - protein, 179 aa, synthetic construct; identical to SEQ ID NO: 317

SEQ ID NO: 320 - DNA, 536 bp, synthetic construct; identical to SEQ ID NO: 318
  source 1..536: mol_type = other DNA

SEQ ID NO: 321 - protein, 179 aa, synthetic construct; identical to SEQ ID NO: 317

SEQ ID NO: 322 - DNA, 536 bp, synthetic construct; identical to SEQ ID NO: 318
  source 1..536: mol_type = other DNA

SEQ ID NO: 323 - protein, 179 aa, synthetic construct; identical to SEQ ID NO: 317

SEQ ID NO: 324 - DNA, 536 bp, synthetic construct; identical to SEQ ID NO: 318
  source 1..536: mol_type = other DNA

SEQ ID NO: 325 - protein, 179 aa, synthetic construct; identical to SEQ ID NO: 317

SEQ ID NO: 326 - DNA, 537 bp, synthetic construct
  source 1..537: mol_type = other DNA
gaggacctgaaaaacgtgttcccacccgaggtcgctgtgtttgagccatcagaagcagagatctcccacacccaaaaggccacactggtgtgcctggccacaggcttctaccccgaccacgtggagctgagctggtgggtgaatgggaaggaggtgcacagtggggtcagcacagacccgcagcccctcaaggagcagcccgccctcaatgactccagatactgcctgtcctcccgcctgagggtctcggccaccttctggcagaacccccgcaaccacttccgctgtcaagtccagttctacgggctctcggagaatgacgagtggacccaggatagggccaaacctgtcacccagatcgtcagcgccgaggcctggggtagagcagactgtggcttcacctccgagtcttaccagcaaggggtcctgtctgccaccatcctctatgagatcttgctagggaaggccaccttgtatgccgtgctggtcagtgccctcgtgctgatggccatggtcaagagaaaggattccagaggc

SEQ ID NO: 327 - protein, 177 aa, synthetic construct
EDLNKVFPPEVAVFEPSEAEISHTQKATLVCLATGFFPDHVELSWWVNGKEVHSGVSTDPQPLKEQPALNDSRYCLSSRLRVSATFWQNPRNHFRCQVQFYGLSENDEWTQDRAKPVTQIVSAEAWGRADCGFTSVSYQQGVLSATILYEILLGKATLYAVLVSALVLMAMVKRKDF

SEQ ID NO: 328 - DNA, 531 bp, synthetic construct
  source 1..531: mol_type = other DNA
gaggacctgaacaaggtgttcccacccgaggtcgctgtgtttgagccatcagaagcagagatctcccacacccaaaaggccacactggtgtgcctggccacaggcttcttccctgaccacgtggagctgagctggtgggtgaatgggaaggaggtgcacagtggggtcagcacggacccgcagcccctcaaggagcagcccgccctcaatgactccagatactgcctgtcctcccgcctgagggtctcggccaccttctggcagaacccccgcaaccacttccgctgtcaagtccagttctacgggctctcggagaatgacgagtggacccaggatagggccaaacccgtcacccagatcgtcagcgccgaggcctggggtagagcagactgtggctttacctcggtgtcctaccagcaaggggtcctgtctgccaccatcctctatgagatcctgctagggaaggccaccctgtatgctgtgctggtcagcgcccttgtgttgatggccatggtcaagagaaaggatttc

SEQ ID NO: 329 - protein, 179 aa, synthetic construct; identical to SEQ ID NO: 317

SEQ ID NO: 330 - DNA, 537 bp, synthetic construct; identical to SEQ ID NO: 326
  source 1..537: mol_type = other DNA

SEQ ID NO: 331 - protein, 179 aa, synthetic construct; identical to SEQ ID NO: 317

SEQ ID NO: 332 - DNA, 537 bp, synthetic construct; identical to SEQ ID NO: 326
  source 1..537: mol_type = other DNA

SEQ ID NO: 333 - protein, 177 aa, synthetic construct; identical to SEQ ID NO: 327

SEQ ID NO: 334 - DNA, 531 bp, synthetic construct; identical to SEQ ID NO: 328
  source 1..531: mol_type = other DNA

SEQ ID NO: 335 - protein, 179 aa, synthetic construct; identical to SEQ ID NO: 317

SEQ ID NO: 336 - DNA, 537 bp, synthetic construct; identical to SEQ ID NO: 326
  source 1..537: mol_type = other DNA

SEQ ID NO: 337 - protein, 177 aa, synthetic construct; identical to SEQ ID NO: 327

SEQ ID NO: 338 - DNA, 531 bp, synthetic construct; identical to SEQ ID NO: 328
  source 1..531: mol_type = other DNA

SEQ ID NO: 339 - protein, 179 aa, synthetic construct; identical to SEQ ID NO: 317

SEQ ID NO: 340 - DNA, 537 bp, synthetic construct; identical to SEQ ID NO: 326
  source 1..537: mol_type = other DNA

SEQ ID NO: 341 - protein, 179 aa, synthetic construct; identical to SEQ ID NO: 317

SEQ ID NO: 342 - DNA, 537 bp, synthetic construct; identical to SEQ ID NO: 326
  source 1..537: mol_type = other DNA

SEQ ID NO: 343 - protein, 179 aa, synthetic construct; identical to SEQ ID NO: 317

SEQ ID NO: 344 - DNA, 537 bp, synthetic construct; identical to SEQ ID NO: 326
  source 1..537: mol_type = other DNA

SEQ ID NO: 345 - protein, 177 aa, synthetic construct; identical to SEQ ID NO: 327

SEQ ID NO: 346 - DNA, 531 bp, synthetic construct; identical to SEQ ID NO: 328
  source 1..531: mol_type = other DNA

SEQ ID NO: 347 - protein, 179 aa, synthetic construct; identical to SEQ ID NO: 317

SEQ ID NO: 348 - DNA, 537 bp, synthetic construct; identical to SEQ ID NO: 326
  source 1..537: mol_type = other DNA

SEQ ID NO: 349 - protein, 297 aa, synthetic construct
DVKVTQSSRYLVKRTGEKVFLECVQDMDHENMFWYRQDPGLGLRLIYFSYDVKMKEKGDIPEGYSVSREKKERFSLILESASTNQTSMYLCASSPPHLASGASTDTQYFGPGTRLTVLEDLKNVFPPEVAVFEPSEAEISHTQKATLVCLATGFYPDHVELSWWVNGKEVHSGVSTDPQPLKEQPALNDSRYCLSSRLRVSATFWQNPRNHFRCQVQFYGLSENDEWTQDRAKPVTQIVSAEAWGRADCGFTSESYQQGVLSATILYEILLGKATLYAVLVSALVLMAMVKRKDSRG

SEQ ID NO: 350 - DNA, 891 bp, synthetic construct
  source 1..891: mol_type = other DNA
gatgtgaaagtaacccagagctcgagatatctagtcaaaaggacgggagagaaagtttttctggaatgtgtccaggatatggaccatgaaaatatgttctggtatcgacaagacccaggtctggggctacggctgatctatttctcatatgatgttaaaatgaaagaaaaaggagatattcctgaggggtacagtgtctctagagagaagaaggagcgcttctccctgattctggagtccgccagcaccaaccagacatctatgtacctctgtgccagcagcccgccgcatttagctagcggggcgagcacagatacgcagtattttggcccaggcacccggctgacagtgctcgaggacctgaaaaacgtgttcccacccgaggtcgctgtgtttgagccatcagaagcagagatctcccacacccaaaaggccacactggtgtgcctggccacaggcttctaccccgaccacgtggagctgagctggtgggtgaatgggaaggaggtgcacagtggggtcagcacagacccgcagcccctcaaggagcagcccgccctcaatgactccagatactgcctgtcctcccgcctgagggtctcggccaccttctggcagaacccccgcaaccacttccgctgtcaagtccagttctacgggctctcggagaatgacgagtggacccaggatagggccaaacctgtcacccagatcgtcagcgccgaggcctggggtagagcagactgtggcttcacctccgagtcttaccagcaaggggtcctgtctgccaccatcctctatgagatcttgctagggaaggccaccttgtatgccgtgctggtcagtgccctcgtgctgatggccatggtcaagagaaaggattccagaggc

SEQ ID NO: 351 - protein, 295 aa, synthetic construct
DSGVTQTPKHLITATGQRVTLRCSPRSGDLSVYWYQQSLDQGLQFLIQYYNGEERAKGNILERFSAQQFPDLHSELNLSSLELGDSALYFCASSPRGGDSILDTQYFGPGTRLTVLEDLKNVFPPEVAVFEPSEAEISHTQKATLVCLATGFYPDHVELSWWVNGKEVHSGVSTDPQPLKEQPALNDSRYCLSSRLRVSATFWQNPRNHFRCQVQFYGLSENDEWTQDRAKPVTQIVSAEAWGRADCGFTSESYQQGVLSATILYEILLGKATLYAVLVSALVLMAMVKRKDSRG

SEQ ID NO: 352 - DNA, 885 bp, synthetic construct
  source 1..885: mol_type = other DNA
gattctggagtcacacaaaccccaaagcacctgatcacagcaactggacagcgagtgacgctgagatgctcccctaggtctggagacctctctgtgtactggtaccaacagagcctggaccagggcctccagttcctcattcagtattataatggagaagagagagcaaaaggaaacattcttgaacgattctccgcacaacagttccctgacttgcactctgaactaaacctgagctctctggagctgggggactcagctttgtatttctgtgccagcagcccgagggggggggactctattttggatacgcagtattttggcccaggcacccggctgacagtgctcgaggacctgaaaaacgtgttcccacccgaggtcgctgtgtttgagccatcagaagcagagatctcccacacccaaaaggccacactggtgtgcctggccacaggcttctaccccgaccacgtggagctgagctggtgggtgaatgggaaggaggtgcacagtggggtcagcacagacccgcagcccctcaaggagcagcccgccctcaatgactccagatactgcctgtcctcccgcctgagggtctcggccaccttctggcagaacccccgcaaccacttccgctgtcaagtccagttctacgggctctcggagaatgacgagtggacccaggatagggccaaacctgtcacccagatcgtcagcgccgaggcctggggtagagcagactgtggcttcacctccgagtcttaccagcaaggggtcctgtctgccaccatcctctatgagatcttgctagggaaggccaccttgtatgccgtgctggtcagtgccctcgtgctgatggccatggtcaagagaaaggattccagaggc

SEQ ID NO: 353 - protein, 292 aa, synthetic construct
EAQVTQNPRYLITVTGKKLTVTCSQNMNHEYMSWYRQDPGLGLRQIYYSMNVEVTDKGDVPEGYKVSRKEKRNFPLILESPSPNQTSLYFCASSTRDRDNEQFFGPGTRLTVLEDLKNVFPPEVAVFEPSEAEISHTQKATLVCLATGFYPDHVELSWWVNGKEVHSGVSTDPQPLKEQPALNDSRYCLSSRLRVSATFWQNPRNHFRCQVQFYGLSENDEWTQDRAKPVTQIVSAEAWGRADCGFTSESYQQGVLSATILYEILLGKATLYAVLVSALVLMAMVKRKDSRG

SEQ ID NO: 354 - DNA, 876 bp, synthetic construct
  source 1..876: mol_type = other DNA
gaagcccaagtgacccagaacccaagatacctcatcacagtgactggaaagaagttaacagtgacttgttctcagaatatgaaccatgagtatatgtcctggtatcgacaagacccagggctgggcttaaggcagatctactattcaatgaatgttgaggtgactgataagggagatgttcctgaagggtacaaagtctctcgaaaagagaagaggaatttccccctgatcctggagtcgcccagccccaaccagacctctctgtacttctgtgccagcagcacccgggacagggacaatgagcagttcttcgggccagggacacggctcaccgtgctagaggacctgaaaaacgtgttcccacccgaggtcgctgtgtttgagccatcagaagcagagatctcccacacccaaaaggccacactggtgtgcctggccacaggcttctaccccgaccacgtggagctgagctggtgggtgaatgggaaggaggtgcacagtggggtcagcacagacccgcagcccctcaaggagcagcccgccctcaatgactccagatactgcctgtcctcccgcctgagggtctcggccaccttctggcagaacccccgcaaccacttccgctgtcaagtccagttctacgggctctcggagaatgacgagtggacccaggatagggccaaacctgtcacccagatcgtcagcgccgaggcctggggtagagcagactgtggcttcacctccgagtcttaccagcaaggggtcctgtctgccaccatcctctatgagatcttgctagggaaggccaccttgtatgccgtgctggtcagtgccctcgtgctgatggccatggtcaagagaaaggattccagaggc

SEQ ID NO: 355 - protein, 293 aa, synthetic construct
DARVTQTPRDKVTEMGQEVTMRCQPILGHNTVFWYRQTMMQGLELLAYFRNRAPLDDSGMPKDRFSAEMPDATLATLKIQPSEPRDSAVYFCASGPEGLDNEQFFGPGTRLTVLEDLKNVFPPEVAVFEPSEAEISHTQKATLVCLATGFYPDHVELSWWVNGKEVHSGVSTDPQPLKEQPALNDSRYCLSSRLRVSATFWQNPRNHFRCQVQFYGLSENDEWTQDRAKPVTQIVSAEAWGRADCGFTSESYQQGVLSATILYEILLGKATLYAVLVSALVLMAMVKRKDSRG

SEQ ID NO: 356 - DNA, 879 bp, synthetic construct
  source 1..879: mol_type = other DNA
gatgctagagtcacccagacaccaagggacaaggtgacagagatgggacaagaagtaacaatgagatgtcagccaattttaggccacaatactgttttctggtacagacagaccatgatgcaaggactggagttgctggcttacttccgcaaccgggctcctctagatgattcggggatgccgaaggatcgattctcagcagagatgcctgatgcaactttagccactctgaagatccagccctcagaacccagggactcagctgtgtatttttgtgctagtggtcccgaggggttggacaatgagcagttcttcgggccagggacacggctcaccgtgctagaggacctgaaaaacgtgttcccacccgaggtcgctgtgtttgagccatcagaagcagagatctcccacacccaaaaggccacactggtgtgcctggccacaggcttctaccccgaccacgtggagctgagctggtgggtgaatgggaaggaggtgcacagtggggtcagcacagacccgcagcccctcaaggagcagcccgccctcaatgactccagatactgcctgtcctcccgcctgagggtctcggccaccttctggcagaacccccgcaaccacttccgctgtcaagtccagttctacgggctctcggagaatgacgagtggacccaggatagggccaaacctgtcacccagatcgtcagcgccgaggcctggggtagagcagactgtggcttcacctccgagtcttaccagcaaggggtcctgtctgccaccatcctctatgagatcttgctagggaaggccaccttgtatgccgtgctggtcagtgccctcgtgctgatggccatggtcaagagaaaggattccagaggc

SEQ ID NO: 357 - protein, 294 aa, synthetic construct
GAVVSQHPSWVICKSGTSVKIECRSLDFQATTMFWYRQFPKQSLMLMATSNEGSKATYEQGVEKDKFLINHASLTLSTLTVTSAHPEDSSFYICSARFANYYEQYFGPGTRLTVTEDLKNVFPPEVAVFEPSEAEISHTQKATLVCLATGFYPDHVELSWWVNGKEVHSGVSTDPQPLKEQPALNDSRYCLSSRLRVSATFWQNPRNHFRCQVQFYGLSENDEWTQDRAKPVTQIVSAEAWGRADCGFTSESYQQGVLSATILYEILLGKATLYAVLVSALVLMAMVKRKDSRG

SEQ ID NO: 358 - DNA, 882 bp, synthetic construct
  source 1..882: mol_type = other DNA
ggtgctgtcgtctctcaacatccgagctgggttatctgtaagagtggaacctctgtgaagatcgagtgccgttccctggactttcaggccacaactatgttttggtatcgtcagttcccgaaacagagtctcatgctgatggcaacttccaatgagggctccaaggccacatacgagcaaggcgtcgagaaggacaagtttctcatcaaccatgcaagcctgaccttgtccactctgacagtgaccagtgcccatcctgaagacagcagcttctacatctgcagtgctaggtttgccaattactacgagcagtacttcgggccgggcaccaggctcacggtcacagaggacctgaaaaacgtgttcccacccgaggtcgctgtgtttgagccatcagaagcagagatctcccacacccaaaaggccacactggtgtgcctggccacaggcttctaccccgaccacgtggagctgagctggtgggtgaatgggaaggaggtgcacagtggggtcagcacagacccgcagcccctcaaggagcagcccgccctcaatgactccagatactgcctgtcctcccgcctgagggtctcggccaccttctggcagaacccccgcaaccacttccgctgtcaagtccagttctacgggctctcggagaatgacgagtggacccaggatagggccaaacctgtcacccagatcgtcagcgccgaggcctggggtagagcagactgtggcttcacctccgagtcttaccagcaaggggtcctgtctgccaccatcctctatgagatcttgctagggaaggccaccttgtatgccgtgctggtcagtgccctcgtgctgatggccatggtcaagagaaaggattccagaggc

SEQ ID NO: 359 - protein, 291 aa, synthetic construct
EADIYQTPRYLVIGTGKKITLECSQTMGHDKMYWYQQDPGMELHLIHYSYGVNSTEKGDLSSESTVSRIRTEHFPLTLESARPSHTSQYLCASSDPVHGDYGYTFGSGTRLTVVEDLNKVFPPEVAVFEPSEAEISHTQKATLVCLATGFFPDHVELSWWVNGKEVHSGVSTDPQPLKEQPALNDSRYCLSSRLRVSATFWQNPRNHFRCQVQFYGLSENDEWTQDRAKPVTQIVSAEAWGRADCGFTSVSYQQGVLSATILYEILLGKATLYAVLVSALVLMAMVKRKDF

SEQ ID NO: 360 - DNA, 873 bp, synthetic construct
  source 1..873: mol_type = other DNA
gaagctgacatctaccagaccccaagataccttgttatagggacaggaaagaagatcactctggaatgttctcaaaccatgggccatgacaaaatgtactggtatcaacaagatccaggaatggaactacacctcatccactattcctatggagttaattccacagagaagggagatctttcctctgagtcaacagtctccagaataaggacggagcattttcccctgaccctggagtctgccaggccctcacatacctctcagtacctctgtgccagcagtgacccagtacacggcgactatggctacaccttcggttcggggaccaggttaaccgttgtagaggacctgaacaaggtgttcccacccgaggtcgctgtgtttgagccatcagaagcagagatctcccacacccaaaaggccacactggtgtgcctggccacaggcttcttccctgaccacgtggagctgagctggtgggtgaatgggaaggaggtgcacagtggggtcagcacggacccgcagcccctcaaggagcagcccgccctcaatgactccagatactgcctgtcctcccgcctgagggtctcggccaccttctggcagaacccccgcaaccacttccgctgtcaagtccagttctacgggctctcggagaatgacgagtggacccaggatagggccaaacccgtcacccagatcgtcagcgccgaggcctggggtagagcagactgtggctttacctcggtgtcctaccagcaaggggtcctgtctgccaccatcctctatgagatcctgctagggaaggccaccctgtatgctgtgctggtcagcgcccttgtgttgatggccatggtcaagagaaaggatttc

SEQ ID NO: 361 - protein, 292 aa, synthetic construct
GEEVAQTPKHLVRGEGQKAKLYCAPIKGHSYVFWYQQVLKNEFKFLISFQNENVFDETGMPKERFSAKCLPNSPCSLEIQATKLEDSAVYFCASSPHHRYEQYFGPGTRLTVTEDLKNVFPPEVAVFEPSEAEISHTQKATLVCLATGFYPDHVELSWWVNGKEVHSGVSTDPQPLKEQPALNDSRYCLSSRLRVSATFWQNPRNHFRCQVQFYGLSENDEWTQDRAKPVTQIVSAEAWGRADCGFTSESYQQGVLSATILYEILLGKATLYAVLVSALVLMAMVKRKDSRG

SEQ ID NO: 362 - DNA, 876 bp, synthetic construct
  source 1..876: mol_type = other DNA
ggtgaagaagtcgcccagactccaaaacatcttgtcagaggggaaggacagaaagcaaaattatattgtgccccaataaaaggacacagttatgttttttggtaccaacaggtcctgaaaaacgagttcaagttcttgatttccttccagaatgaaaatgtctttgatgaaacaggtatgcccaaggaaagattttcagctaagtgcctcccaaattcaccctgtagccttgagatccaggctacgaagcttgaggattcagcagtgtatttttgtgccagcagcccacaccacaggtacgagcagtacttcgggccgggcaccaggctcacggtcacagaggacctgaaaaacgtgttcccacccgaggtcgctgtgtttgagccatcagaagcagagatctcccacacccaaaaggccacactggtgtgcctggccacaggcttctaccccgaccacgtggagctgagctggtgggtgaatgggaaggaggtgcacagtggggtcagcacagacccgcagcccctcaaggagcagcccgccctcaatgactccagatactgcctgtcctcccgcctgagggtctcggccaccttctggcagaacccccgcaaccacttccgctgtcaagtccagttctacgggctctcggagaatgacgagtggacccaggatagggccaaacctgtcacccagatcgtcagcgccgaggcctggggtagagcagactgtggcttcacctccgagtcttaccagcaaggggtcctgtctgccaccatcctctatgagatcttgctagggaaggccaccttgtatgccgtgctggtcagtgccctcgtgctgatggccatggtcaagagaaaggattccagaggc

SEQ ID NO: 363 - protein, 291 aa, synthetic construct
EAQVTQNPRYLITVTGKKLTVTCSQNMNHEYMSWYRQDPGLGLRQIYYSMNVEVTDKGDVPEGYKVSRKEKRNFPLILESPSPNQTSLYFCASSTSPYNEQFFGPGTRLTVLEDLKNVFPPEVAVFEPSEAEISHTQKATLVCLATGFYPDHVELSWWVNGKEVHSGVSTDPQPLKEQPALNDSRYCLSSRLRVSATFWQNPRNHFRCQVQFYGLSENDEWTQDRAKPVTQIVSAEAWGRADCGFTSESYQQGVLSATILYEILLGKATLYAVLVSALVLMAMVKRKDSRG

SEQ ID NO: 364 - DNA, 873 bp, synthetic construct
  source 1..873: mol_type = other DNA
gaagcccaagtgacccagaacccaagatacctcatcacagtgactggaaagaagttaacagtgacttgttctcagaatatgaaccatgagtatatgtcctggtatcgacaagacccagggctgggcttaaggcagatctactattcaatgaatgttgaggtgactgataagggagatgttcctgaagggtacaaagtctctcgaaaagagaagaggaatttccccctgatcctggagtcgcccagccccaaccagacctctctgtacttctgtgccagctcgactagcccgtacaatgagcagttcttcgggccagggacacggctcaccgtgctagaggacctgaaaaacgtgttcccacccgaggtcgctgtgtttgagccatcagaagcagagatctcccacacccaaaaggccacactggtgtgcctggccacaggcttctaccccgaccacgtggagctgagctggtgggtgaatgggaaggaggtgcacagtggggtcagcacagacccgcagcccctcaaggagcagcccgccctcaatgactccagatactgcctgtcctcccgcctgagggtctcggccaccttctggcagaacccccgcaaccacttccgctgtcaagtccagttctacgggctctcggagaatgacgagtggacccaggatagggccaaacctgtcacccagatcgtcagcgccgaggcctggggtagagcagactgtggcttcacctccgagtcttaccagcaaggggtcctgtctgccaccatcctctatgagatcttgctagggaaggccaccttgtatgccgtgctggtcagtgccctcgtgctgatggccatggtcaagagaaaggattccagaggc

SEQ ID NO: 365 - protein, 291 aa, synthetic construct
DSGVTQTPKHLITATGQRVTLRCSPRSGDLSVYWYQQSLDQGLQFLIQYYNGEERAKGNILERFSAQQFPDLHSELNLSSLELGDSALYFCASSLHRDSDTEAFFGQGTRLTVVEDLNKVFPPEVAVFEPSEAEISHTQKATLVCLATGFFPDHVELSWWVNGKEVHSGVSTDPQPLKEQPALNDSRYCLSSRLRVSATFWQNPRNHFRCQVQFYGLSENDEWTQDRAKPVTQIVSAEAWGRADCGFTSVSYQQGVLSATILYEILLGKATLYAVLVSALVLMAMVKRKDF

SEQ ID NO: 366 - DNA, 873 bp, synthetic construct
  source 1..873: mol_type = other DNA
gattctggagtcacacaaaccccaaagcacctgatcacagcaactggacagcgagtgacgctgagatgctcccctaggtctggagacctctctgtgtactggtaccaacagagcctggaccagggcctccagttcctcattcagtattataatggagaagagagagcaaaaggaaacattcttgaacgattctccgcacaacagttccctgacttgcactctgaactaaacctgagctctctggagctgggggactcagctttgtatttctgtgccagcagcctacaccgggacagtgacactgaagctttctttggacaaggcaccagactcacagttgtagaggacctgaacaaggtgttcccacccgaggtcgctgtgtttgagccatcagaagcagagatctcccacacccaaaaggccacactggtgtgcctggccacaggcttcttccctgaccacgtggagctgagctggtgggtgaatgggaaggaggtgcacagtggggtcagcacggacccgcagcccctcaaggagcagcccgccctcaatgactccagatactgcctgtcctcccgcctgagggtctcggccaccttctggcagaacccccgcaaccacttccgctgtcaagtccagttctacgggctctcggagaatgacgagtggacccaggatagggccaaacccgtcacccagatcgtcagcgccgaggcctggggtagagcagactgtggctttacctcggtgtcctaccagcaaggggtcctgtctgccaccatcctctatgagatcctgctagggaaggccaccctgtatgctgtgctggtcagcgcccttgtgttgatggccatggtcaagagaaaggatttc

SEQ ID NO: 367 - protein, 293 aa, synthetic construct
DSGVTQTPKHLITATGQRVTLRCSPRSGDLSVYWYQQSLDQGLQFLIQYYNGEERAKGNILERFSAQQFPDLHSELNLSSLELGDSALYFCASSHGRDSTDTQYFGPGTRLTVLEDLKNVFPPEVAVFEPSEAEISHTQKATLVCLATGFYPDHVELSWWVNGKEVHSGVSTDPQPLKEQPALNDSRYCLSSRLRVSATFWQNPRNHFRCQVQFYGLSENDEWTQDRAKPVTQIVSAEAWGRADCGFTSESYQQGVLSATILYEILLGKATLYAVLVSALVLMAMVKRKDSRG

SEQ ID NO: 368 - DNA, 879 bp, synthetic construct
  source 1..879: mol_type = other DNA
gattctggagtcacacaaaccccaaagcacctgatcacagcaactggacagcgagtgacgctgagatgctcccctaggtctggagacctctctgtgtactggtaccaacagagcctggaccagggcctccagttcctcattcagtattataatggagaagagagagcaaaaggaaacattcttgaacgattctccgcacaacagttccctgacttgcactctgaactaaacctgagctctctggagctgggggactcagctttgtatttctgtgccagcagccacgggagggatagcacagatacgcagtattttggcccaggcacccggctgacagtgctcgaggacctgaaaaacgtgttcccacccgaggtcgctgtgtttgagccatcagaagcagagatctcccacacccaaaaggccacactggtgtgcctggccacaggcttctaccccgaccacgtggagctgagctggtgggtgaatgggaaggaggtgcacagtggggtcagcacagacccgcagcccctcaaggagcagcccgccctcaatgactccagatactgcctgtcctcccgcctgagggtctcggccaccttctggcagaacccccgcaaccacttccgctgtcaagtccagttctacgggctctcggagaatgacgagtggacccaggatagggccaaacctgtcacccagatcgtcagcgccgaggcctggggtagagcagactgtggcttcacctccgagtcttaccagcaaggggtcctgtctgccaccatcctctatgagatcttgctagggaaggccaccttgtatgccgtgctggtcagtgccctcgtgctgatggccatggtcaagagaaaggattccagaggc

SEQ ID NO: 369 - protein, 290 aa, synthetic construct
GAGVSQSPSNKVTEKGKDVELRCDPISGHTALYWYRQRLGQGLEFLIYFQGNSAPDKSGLPSDRFSAERTGESVSTLTIQRTQQEDSAVYLCASSPGGNYGYTFGSGTRLTVVEDLNKVFPPEVAVFEPSEAEISHTQKATLVCLATGFFPDHVELSWWVNGKEVHSGVSTDPQPLKEQPALNDSRYCLSSRLRVSATFWQNPRNHFRCQVQFYGLSENDEWTQDRAKPVTQIVSAEAWGRADCGFTSVSYQQGVLSATILYEILLGKATLYAVLVSALVLMAMVKRKDF

SEQ ID NO: 370 - DNA, 870 bp, synthetic construct
  source 1..870: mol_type = other DNA
ggagctggagtctcccagtcccccagtaacaaggtcacagagaagggaaaggatgtagagctcaggtgtgatccaatttcaggtcatactgccctttactggtaccgacagaggctggggcagggcctggagtttttaatttacttccaaggcaacagtgcaccagacaaatcagggctgcccagtgatcgcttctctgcagagaggactggggaatccgtctccactctgacgatccagcgcacacagcaggaggactcggccgtgtatctctgtgccagctccccgggggggaactatggctacaccttcggttcggggaccaggttaaccgttgtagaggacctgaacaaggtgttcccacccgaggtcgctgtgtttgagccatcagaagcagagatctcccacacccaaaaggccacactggtgtgcctggccacaggcttcttccctgaccacgtggagctgagctggtgggtgaatgggaaggaggtgcacagtggggtcagcacggacccgcagcccctcaaggagcagcccgccctcaatgactccagatactgcctgtcctcccgcctgagggtctcggccaccttctggcagaacccccgcaaccacttccgctgtcaagtccagttctacgggctctcggagaatgacgagtggacccaggatagggccaaacccgtcacccagatcgtcagcgccgaggcctggggtagagcagactgtggctttacctcggtgtcctaccagcaaggggtcctgtctgccaccatcctctatgagatcctgctagggaaggccaccctgtatgctgtgctggtcagcgcccttgtgttgatggccatggtcaagagaaaggatttc

SEQ ID NO: 371 - protein, 290 aa, synthetic construct
DSGVTQTPKHLITATGQRVTLRCSPRSGDLSVYWYQQSLDQGLQFLIQYYNGEERAKGNILERFSAQQFPDLHSELNLSSLELGDSALYFCASSLGDSEQFFGPGTRLTVLEDLKNVFPPEVAVFEPSEAEISHTQKATLVCLATGFYPDHVELSWWVNGKEVHSGVSTDPQPLKEQPALNDSRYCLSSRLRVSATFWQNPRNHFRCQVQFYGLSENDEWTQDRAKPVTQIVSAEAWGRADCGFTSESYQQGVLSATILYEILLGKATLYAVLVSALVLMAMVKRKDSRG

SEQ ID NO: 372 - DNA, 870 bp, synthetic construct
  source 1..870: mol_type = other DNA
gattctggagtcacacaaaccccaaagcacctgatcacagcaactggacagcgagtgacgctgagatgctcccctaggtctggagacctctctgtgtactggtaccaacagagcctggaccagggcctccagttcctcattcagtattataatggagaagagagagcaaaaggaaacattcttgaacgattctccgcacaacagttccctgacttgcactctgaactaaacctgagctctctggagctgggggactcagctttgtatttctgtgccagcagcctcggggacagcgagcagttcttcgggccagggacacggctcaccgtgctagaggacctgaaaaacgtgttcccacccgaggtcgctgtgtttgagccatcagaagcagagatctcccacacccaaaaggccacactggtgtgcctggccacaggcttctaccccgaccacgtggagctgagctggtgggtgaatgggaaggaggtgcacagtggggtcagcacagacccgcagcccctcaaggagcagcccgccctcaatgactccagatactgcctgtcctcccgcctgagggtctcggccaccttctggcagaacccccgcaaccacttccgctgtcaagtccagttctacgggctctcggagaatgacgagtggacccaggatagggccaaacctgtcacccagatcgtcagcgccgaggcctggggtagagcagactgtggcttcacctccgagtcttaccagcaaggggtcctgtctgccaccatcctctatgagatcttgctagggaaggccaccttgtatgccgtgctggtcagtgccctcgtgctgatggccatggtcaagagaaaggattccagaggc

SEQ ID NO: 373 - protein, 295 aa, synthetic construct
GAGVSQSPSNKVTEKGKDVELRCDPISGHTALYWYRQSLGQGLEFLIYFQGNSAPDKSGLPSDRFSAERTGGSVSTLTIQRTQQEDSAVYLCASSFGTSGDQYEQYFGPGTRLTVTEDLKNVFPPEVAVFEPSEAEISHTQKATLVCLATGFYPDHVELSWWVNGKEVHSGVSTDPQPLKEQPALNDSRYCLSSRLRVSATFWQNPRNHFRCQVQFYGLSENDEWTQDRAKPVTQIVSAEAWGRADCGFTSESYQQGVLSATILYEILLGKATLYAVLVSALVLMAMVKRKDSRG

SEQ ID NO: 374 - DNA, 885 bp, synthetic construct
  source 1..885: mol_type = other DNA
ggagctggagtctcccagtcccccagtaacaaggtcacagagaagggaaaggatgtagagctcaggtgtgatccaatttcaggtcatactgccctttactggtaccgacagagcctggggcagggcctggagtttttaatttacttccaaggcaacagtgcaccagacaaatcagggctgcccagtgatcgcttctctgcagagaggactgggggatccgtctccactctgacgatccagcgcacacagcaggaggactcggccgtgtatctctgtgccagcagctttgggactagcggggaccaatacgagcagtacttcgggccgggcaccaggctcacggtcacagaggacctgaaaaacgtgttcccacccgaggtcgctgtgtttgagccatcagaagcagagatctcccacacccaaaaggccacactggtgtgcctggccacaggcttctaccccgaccacgtggagctgagctggtgggtgaatgggaaggaggtgcacagtggggtcagcacagacccgcagcccctcaaggagcagcccgccctcaatgactccagatactgcctgtcctcccgcctgagggtctcggccaccttctggcagaacccccgcaaccacttccgctgtcaagtccagttctacgggctctcggagaatgacgagtggacccaggatagggccaaacctgtcacccagatcgtcagcgccgaggcctggggtagagcagactgtggcttcacctccgagtcttaccagcaaggggtcctgtctgccaccatcctctatgagatcttgctagggaaggccaccttgtatgccgtgctggtcagtgccctcgtgctgatggccatggtcaagagaaaggattccagaggc

SEQ ID NO: 375 - protein, 291 aa, synthetic construct
ETGVTQSPTHLIKTRGQQVTLRCSSQSGHNTVSWYQQALGQGPQFIFQYYREEENGRGNFPPRFSGLQFPNYSSELNVNALELDDSALYLCASSLQTGDEQYFGPGTRLTVTEDLKNVFPPEVAVFEPSEAEISHTQKATLVCLATGFYPDHVELSWWVNGKEVHSGVSTDPQPLKEQPALNDSRYCLSSRLRVSATFWQNPRNHFRCQVQFYGLSENDEWTQDRAKPVTQIVSAEAWGRADCGFTSESYQQGVLSATILYEILLGKATLYAVLVSALVLMAMVKRKDSRG

SEQ ID NO: 376 - DNA, 873 bp, synthetic construct
  source 1..873: mol_type = other DNA
gagactggagtcacccaaagtcccacacacctgatcaaaacgagaggacagcaagtgactctgagatgctcttctcagtctgggcacaacactgtgtcctggtaccaacaggccctgggtcaggggccccagtttatctttcagtattatagggaggaagagaatggcagaggaaacttccctcctagattctcaggtctccagttccctaattatagctctgagctgaatgtgaacgccttggagctggacgactcggccctgtatctctgtgccagcagcctgcagacaggggacgagcagtacttcgggccgggcaccaggctcacggtcacagaggacctgaaaaacgtgttcccacccgaggtcgctgtgtttgagccatcagaagcagagatctcccacacccaaaaggccacactggtgtgcctggccacaggcttctaccccgaccacgtggagctgagctggtgggtgaatgggaaggaggtgcacagtggggtcagcacagacccgcagcccctcaaggagcagcccgccctcaatgactccagatactgcctgtcctcccgcctgagggtctcggccaccttctggcagaacccccgcaaccacttccgctgtcaagtccagttctacgggctctcggagaatgacgagtggacccaggatagggccaaacctgtcacccagatcgtcagcgccgaggcctggggtagagcagactgtggcttcacctccgagtcttaccagcaaggggtcctgtctgccaccatcctctatgagatcttgctagggaaggccaccttgtatgccgtgctggtcagtgccctcgtgctgatggccatggtcaagagaaaggattccagaggc

SEQ ID NO: 377 - protein, 291 aa, synthetic construct
EAQVTQNPRYLITVTGKKLTVTCSQNMNHEYMSWYRQDPGLGLRQIYYSMNVEVTDKGDVPEGYKVSRKEKRNFPLILESPSPNQTSLYFCASSSGTGGGAEAFFGQGTRLTVVEDLNKVFPPEVAVFEPSEAEISHTQKATLVCLATGFFPDHVELSWWVNGKEVHSGVSTDPQPLKEQPALNDSRYCLSSRLRVSATFWQNPRNHFRCQVQFYGLSENDEWTQDRAKPVTQIVSAEAWGRADCGFTSVSYQQGVLSATILYEILLGKATLYAVLVSALVLMAMVKRKDF

SEQ ID NO: 378 - DNA, 873 bp, synthetic construct
  source 1..873: mol_type = other DNA
gaagcccaagtgacccagaacccaagatacctcatcacagtgactggaaagaagttaacagtgacttgttctcagaatatgaaccatgagtatatgtcctggtatcgacaagacccagggctgggcttaaggcagatctactattcaatgaatgttgaggtgactgataagggagatgttcctgaagggtacaaagtctctcgaaaagagaagaggaatttccccctgatcctggagtcgcccagccccaaccagacctctctgtacttctgtgccagcagttccgggacagggggtggggctgaagctttctttggacaaggcaccagactcacagttgtagaggacctgaacaaggtgttcccacccgaggtcgctgtgtttgagccatcagaagcagagatctcccacacccaaaaggccacactggtgtgcctggccacaggcttcttccctgaccacgtggagctgagctggtgggtgaatgggaaggaggtgcacagtggggtcagcacggacccgcagcccctcaaggagcagcccgccctcaatgactccagatactgcctgtcctcccgcctgagggtctcggccaccttctggcagaacccccgcaaccacttccgctgtcaagtccagttctacgggctctcggagaatgacgagtggacccaggatagggccaaacccgtcacccagatcgtcagcgccgaggcctggggtagagcagactgtggctttacctcggtgtcctaccagcaaggggtcctgtctgccaccatcctctatgagatcctgctagggaaggccaccctgtatgctgtgctggtcagcgcccttgtgttgatggccatggtcaagagaaaggatttc

SEQ ID NO: 379 - protein, 295 aa, synthetic construct
GAVVSQHPSWVICKSGTSVKIECRSLDFQATTMFWYRQFPKQSLMLMATSNEGSKATYEQGVEKDKFLINHASLTLSTLTVTSAHPEDSSFYICSANRDFGIYEQYFGPGTRLTVTEDLKNVFPPEVAVFEPSEAEISHTQKATLVCLATGFYPDHVELSWWVNGKEVHSGVSTDPQPLKEQPALNDSRYCLSSRLRVSATFWQNPRNHFRCQVQFYGLSENDEWTQDRAKPVTQIVSAEAWGRADCGFTSESYQQGVLSATILYEILLGKATLYAVLVSALVLMAMVKRKDSRG

SEQ ID NO: 380 - DNA, 885 bp, synthetic construct
  source 1..885: mol_type = other DNA
ggtgctgtcgtctctcaacatccgagctgggttatctgtaagagtggaacctctgtgaagatcgagtgccgttccctggactttcaggccacaactatgttttggtatcgtcagttcccgaaacagagtctcatgctgatggcaacttccaatgagggctccaaggccacatacgagcaaggcgtcgagaaggacaagtttctcatcaaccatgcaagcctgaccttgtccactctgacagtgaccagtgcccatcctgaagacagcagcttctacatctgcagtgcgaaccgggacttcgggatctacgagcagtacttcgggccgggcaccaggctcacggtcacagaggacctgaaaaacgtgttcccacccgaggtcgctgtgtttgagccatcagaagcagagatctcccacacccaaaaggccacactggtgtgcctggccacaggcttctaccccgaccacgtggagctgagctggtgggtgaatgggaaggaggtgcacagtggggtcagcacagacccgcagcccctcaaggagcagcccgccctcaatgactccagatactgcctgtcctcccgcctgagggtctcggccaccttctggcagaacccccgcaaccacttccgctgtcaagtccagttctacgggctctcggagaatgacgagtggacccaggatagggccaaacctgtcacccagatcgtcagcgccgaggcctggggtagagcagactgtggcttcacctccgagtcttaccagcaaggggtcctgtctgccaccatcctctatgagatcttgctagggaaggccaccttgtatgccgtgctggtcagtgccctcgtgctgatggccatggtcaagagaaaggattccagaggc

SEQ ID NO: 381 - protein, 10 aa, synthetic construct
VVVGAVGVGK

SEQ ID NO: 382 - protein, 9 aa, synthetic construct
VVGAVGVGK

SEQ ID NO: 383 - DNA, 20 bp, synthetic construct
  source 1..20: mol_type = other DNA
tcagggttctggatatctgt

SEQ ID NO: 384 - DNA, 20 bp, synthetic construct
  source 1..20: mol_type = other DNA
ctgcctgagcagccgcctga

SEQ ID NO: 385 - skipped

SEQ ID NO: 386 - DNA, 3135 bp, synthetic construct
  source 1..3135: mol_type = other DNA
ccatattctggcagggtcagtggctccaactaacatttgtttggtactttacagtttattaaatagatgtttatatggagaagctctcatttctttctcagaagagcctggctaggaaggtggatgaggcaccatattcattttgcaggtgaaattcctgagatgtaaggagctgctgtgacttgctcaaggccttatatcgagtaaacggtagtgctggggcttagacgcaggtgttctgatttatagttcaaaacctctatcaatgagagagcaatctcctggtaatgtgatagatttcccaacttaatgccaacataccataaacctcccattctgctaatgcccagcctaagttggggagaccactccagattccaagatgtacagtttgctttgctgggcctttttcccatgcctgcctttactctgccagagttatattgctggggttttgaagaagatcctattaaataaaagaataagcagtattattaagtagccctgcatttcaggtttccttgagtggcaggccaggcctggccgtgaacgttcactgaaatcatggcctcttggccaagattgatagcttgtgcctgtccctgagtcccagtccatcacgagcagctggtttctaagatgctatttcccgtataaagcatgagaccgtgacttgccagccccacagagccccgcccttgtccatcactggcatctggactccagcctgggttggggcaaagagggaaatgagatcatgtcctaaccctgatcctcttgtcccacagatggcagcggcgccaccaacttcagcctgctgaagcaggccggcgacgtggaggagaaccccggccccatggccaccggcagcaggaccagcctgctgctggccttcggcctgctgtgcctgccctggctgcaggagggcagcgccgattctggagtcacacaaaccccaaagcacctgatcacagcaactggacagcgagtgacgctgagatgctcccctaggtctggagacctctctgtgtactggtaccaacagagcctggaccagggcctccagttcctcattcagtattataatggagaagagagagcaaaaggaaacattcttgaacgattctccgcacaacagttccctgacttgcactctgaactaaacctgagctctctggagctgggggactcagctttgtatttctgtgccagcagcccgagggggggggactctattttggatacgcagtattttggcccaggcacccggctgacagtgctcgaggacctgaaaaacgtgttcccacccgaggtcgctgtgtttgagccatcagaagcagagatctcccacacccaaaaggccacactggtgtgcctggccacaggcttctaccccgaccacgtggagctgagctggtgggtgaatgggaaggaggtgcacagtggggtcagcacagacccgcagcccctcaaggagcagcccgccctcaatgactccagatactgcctgtcctcccgcctgagggtctcggccaccttctggcagaacccccgcaaccacttccgctgtcaagtccagttctacgggctctcggagaatgacgagtggacccaggatagggccaaacctgtcacccagatcgtcagcgccgaggcctggggtagagcagactgtggcttcacctccgagtcttaccagcaaggggtcctgtctgccaccatcctctatgagatcttgctagggaaggccaccttgtatgccgtgctggtcagtgccctcgtgctgatggccatggtcaagagaaaggattccagaggccgggccaagcggggatccggagccacaaatttctccctgctgaaacaggccggcgatgtggaggagaatcctggacctatggccaccggcagcaggaccagcctgctgctggccttcggcctgctgtgcctgccctggctgcaggagggcagcgccgctcagaaggtaactcaagcgcagactgaaatttctgtggtggagaaggaggatgtgaccttggactgtgtgtatgaaacccgtgatactacttattacttattctggtacaagcaaccaccaagtggagaattggttttccttattcgtcggaactcttttgatgagcaaaatgaaataagtggtcggtattcttggaacttccagaaatccaccagttccttcaacttcaccatcacagcctcacaagtcgtggactcagcagtatacttctgtgctctgagtgacccccgttattcaggaggaggtgctgacggactcacctttggcaaagggactcatctaatcatccagccctatatccagaaccctgaccctgccgtgtaccagctgagagactctaaatccagtgacaagtctgtctgcctattcaccgattttgattctcaaacaaatgtgtcacaaagtaaggattctgatgtgtatatcacagacaaaactgtgctagacatgaggtctatggacttcaagagcaacagtgctgtggcctggagcaacaaatctgactttgcatgtgcaaacgccttcaacaacagcattattccagaagacaccttcttccccagcccaggtaagggcagctttggtgccttcgcaggctgtttccttgcttcaggaatggccaggttctgcccagagctctggtcaatgatgtctaaaactcctctgattggtggtctcggccttatccattgccaccaaaaccctctttttactaagaaacagtgagccttgttctggcagtccagagaatgacacgggaaaaaagcagatgaagagaaggtggcaggagagggcacgtggcccagcctcagtctctccaactgagttcctgcctgcctgcctttgctcagactgtttgccccttactgctcttctaggcctcattctaagccccttctccaagttgcctctccttatttctccctgtctgccaaaaaatctttcccagctcactaagtcagtctcacgcagtcactcattaacccaccaatcactgattgtgccggcacatgaatgcaccaggtgttgaagtggaggaattaaaaagtcagatgaggggtgtgcccagaggaagcaccattctagttgggggagcc

SEQ ID NO: 387 - DNA, 790 bp, synthetic construct
  source 1..790: mol_type = other DNA
ccatattctggcagggtcagtggctccaactaacatttgtttggtactttacagtttattaaatagatgtttatatggagaagctctcatttctttctcagaagagcctggctaggaaggtggatgaggcaccatattcattttgcaggtgaaattcctgagatgtaaggagctgctgtgacttgctcaaggccttatatcgagtaaacggtagtgctggggcttagacgcaggtgttctgatttatagttcaaaacctctatcaatgagagagcaatctcctggtaatgtgatagatttcccaacttaatgccaacataccataaacctcccattctgctaatgcccagcctaagttggggagaccactccagattccaagatgtacagtttgctttgctgggcctttttcccatgcctgcctttactctgccagagttatattgctggggttttgaagaagatcctattaaataaaagaataagcagtattattaagtagccctgcatttcaggtttccttgagtggcaggccaggcctggccgtgaacgttcactgaaatcatggcctcttggccaagattgatagcttgtgcctgtccctgagtcccagtccatcacgagcagctggtttctaagatgctatttcccgtataaagcatgagaccgtgacttgccagccccacagagccccgcccttgtccatcactggcatctggactccagcctgggttggggcaaagagggaaatgagatcatgtcctaaccctgatcctcttgtcccacagat

SEQ ID NO: 388 - DNA, 66 bp, synthetic construct
  source 1..66: mol_type = other DNA
ggcagcggcgccaccaacttcagcctgctgaagcaggccggcgacgtggaggagaaccccggcccc

SEQ ID NO: 389 - DNA, 78 bp, synthetic construct
  source 1..78: mol_type = other DNA
atggccaccggcagcaggaccagcctgctgctggccttcggcctgctgtgcctgccctggctgcaggagggcagcgcc

SEQ ID NO: 390 - DNA, 78 bp, synthetic construct
  source 1..78: mol_type = other DNA
cgggccaagcggggatccggagccacaaatttctccctgctgaaacaggccggcgatgtggaggagaatcctggacct

SEQ ID NO: 391 - DNA, 800 bp, synthetic construct
  source 1..800: mol_type = other DNA
atccagaaccctgaccctgccgtgtaccagctgagagactctaaatccagtgacaagtctgtctgcctattcaccgattttgattctcaaacaaatgtgtcacaaagtaaggattctgatgtgtatatcacagacaaaactgtgctagacatgaggtctatggacttcaagagcaacagtgctgtggcctggagcaacaaatctgactttgcatgtgcaaacgccttcaacaacagcattattccagaagacaccttcttccccagcccaggtaagggcagctttggtgccttcgcaggctgtttccttgcttcaggaatggccaggttctgcccagagctctggtcaatgatgtctaaaactcctctgattggtggtctcggccttatccattgccaccaaaaccctctttttactaagaaacagtgagccttgttctggcagtccagagaatgacacgggaaaaaagcagatgaagagaaggtggcaggagagggcacgtggcccagcctcagtctctccaactgagttcctgcctgcctgcctttgctcagactgtttgccccttactgctcttctaggcctcattctaagccccttctccaagttgcctctccttatttctccctgtctgccaaaaaatctttcccagctcactaagtcagtctcacgcagtcactcattaacccaccaatcactgattgtgccggcacatgaatgcaccaggtgttgaagtggaggaattaaaaagtcagatgaggggtgtgcccagaggaagcaccattctagttgggggagcc

SEQ ID NO: 392 - protein, 504 aa, synthetic construct
GSGATNFSLLKQAGDVEENPGPMATGSRTSLLLAFGLLCLPWLQEGSADARVTQTPRDKVTEMGQEVTMRCQPILGHNTVFWYRQTMMQGLELLAYFRNRAPLDDSGMPKDRFSAEMPDATLATLKIQPSEPRDSAVYFCASGPEGLDNEQFFGPGTRLTVLEDLKNVFPPEVAVFEPSEAEISHTQKATLVCLATGFYPDHVELSWWVNGKEVHSGVSTDPQPLKEQPALNDSRYCLSSRLRVSATFWQNPRNHFRCQVQFYGLSENDEWTQDRAKPVTQIVSAEAWGRADCGFTSESYQQGVLSATILYEILLGKATLYAVLVSALVLMAMVKRKDSRGRAKRGSGATNFSLLKQAGDVEENPGPMATGSRTSLLLAFGLLCLPWLQEGSAQKEVEQNSGPLSVPEGAIASLNCTYSDRGSQSFFWYRQYSGKSPELIMFIYSNGDKEDGRFTAQLNKASQYVSLLIRDSQPSDSATYLCAVNMPGNMLTFGGGTRLMVKPH

SEQ ID NO: 393 - DNA, 1512 bp, synthetic construct
  source 1..1512: mol_type = other DNA
ggcagcggcgccaccaacttcagcctgctgaagcaggccggcgacgtggaggagaaccccggccccatggccaccggcagcaggaccagcctgctgctggccttcggcctgctgtgcctgccctggctgcaggagggcagcgccgatgctagagtcacccagacaccaagggacaaggtgacagagatgggacaagaagtaacaatgagatgtcagccaattttaggccacaatactgttttctggtacagacagaccatgatgcaaggactggagttgctggcttacttccgcaaccgggctcctctagatgattcggggatgccgaaggatcgattctcagcagagatgcctgatgcaactttagccactctgaagatccagccctcagaacccagggactcagctgtgtatttttgtgctagtggtcccgaggggttggacaatgagcagttcttcgggccagggacacggctcaccgtgctagaggacctgaaaaacgtgttcccacccgaggtcgctgtgtttgagccatcagaagcagagatctcccacacccaaaaggccacactggtgtgcctggccacaggcttctaccccgaccacgtggagctgagctggtgggtgaatgggaaggaggtgcacagtggggtcagcacagacccgcagcccctcaaggagcagcccgccctcaatgactccagatactgcctgtcctcccgcctgagggtctcggccaccttctggcagaacccccgcaaccacttccgctgtcaagtccagttctacgggctctcggagaatgacgagtggacccaggatagggccaaacctgtcacccagatcgtcagcgccgaggcctggggtagagcagactgtggcttcacctccgagtcttaccagcaaggggtcctgtctgccaccatcctctatgagatcttgctagggaaggccaccttgtatgccgtgctggtcagtgccctcgtgctgatggccatggtcaagagaaaggattccagaggccgggccaagcggggatccggagccacaaatttctccctgctgaaacaggccggcgatgtggaggagaatcctggacctatggccaccggcagcaggaccagcctgctgctggccttcggcctgctgtgcctgccctggctgcaggagggcagcgcccagaaggaggtggagcagaattctggacccctcagtgttccagagggagccattgcctctctcaactgcacttacagtgaccgaggttcccagtccttcttctggtacagacaatattctgggaaaagccctgagttgataatgttcatatactccaatggtgacaaagaagatggaaggtttacagcacagctcaataaagccagccagtatgtttctctgctcatcagagactcccagcccagtgattcagccacctacctctgtgccgtgaacatgccaggcaacatgctcacctttggagggggaacaaggttaatggtcaaaccccat

SEQ ID NO: 394 - protein, 764 aa, synthetic construct
GSGATNFSLLKQAGDVEENPGPMALPVTALLLPLALLLHAARPSQFRVSPLDRTWNLGETVELKCQVLLSNPTSGCSWLFQPRGAAASPTFLLYLSQNKPKAAEGLDTQRFSGKRLGDTFVLTLSDFRRENEGYYFCSALSNSIMYFSHFVPVFLPAKPTTTPAPRPPTPAPTIASQPLSLRPEACRPAAGGAVHTRGLDFACDIYIWAPLAGTCGVLLLSLVITLYCNHRNRRRVCKCPRPVVKSGDKPSLSARYVRAKRGSGEGRGSLLTCGDVEENPGPMATGSRTSLLLAFGLLCLPWLQEGSADARVTQTPRDKVTEMGQEVTMRCQPILGHNTVFWYRQTMMQGLELLAYFRNRAPLDDSGMPKDRFSAEMPDATLATLKIQPSEPRDSAVYFCASGPEGLDNEQFFGPGTRLTVLEDLKNVFPPEVAVFEPSEAEISHTQKATLVCLATGFYPDHVELSWWVNGKEVHSGVSTDPQPLKEQPALNDSRYCLSSRLRVSATFWQNPRNHFRCQVQFYGLSENDEWTQDRAKPVTQIVSAEAWGRADCGFTSESYQQGVLSATILYEILLGKATLYAVLVSALVLMAMVKRKDSRGRAKRGSGATNFSLLKQAGDVEENPGPMATGSRTSLLLAFGLLCLPWLQEGSAQKEVEQNSGPLSVPEGAIASLNCTYSDRGSQSFFWYRQYSGKSPELIMFIYSNGDKEDGRFTAQLNKASQYVSLLIRDSQPSDSATYLCAVNMPGNMLTFGGGTRLMVKPH

SEQ ID NO: 395 - DNA, 2292 bp, synthetic construct
  source 1..2292: mol_type = other DNA
ggcagcggcgccaccaacttcagcctgctgaagcaggccggcgacgtggaggagaaccccggccccatggccttaccagtgaccgccttgctcctgccgctggccttgctgctccacgccgccaggccgagccagttccgggtgtcgccgctggatcggacctggaacctgggcgagacagtggagctgaagtgccaggtgctgctgtccaacccgacgtcgggctgctcgtggctcttccagccgcgcggcgccgccgccagtcccaccttcctcctatacctctcccaaaacaagcccaaggcggccgaggggctggacacccagcggttctcgggcaagaggttgggggacaccttcgtcctcaccctgagcgacttccgccgagagaacgagggctactatttctgctcggccctgagcaactccatcatgtacttcagccacttcgtgccggtcttcctgccagcgaagcccaccacgacgccagcgccgcgaccaccaacaccggcgcccaccatcgcgtcgcagcccctgtccctgcgcccagaggcgtgccggccagcggcggggggcgcagtgcacacgagggggctggacttcgcctgtgatatctacatctgggcgcccttggccgggacttgtggggtccttctcctgtcactggttatcaccctttactgcaaccacaggaaccgaagacgtgtttgcaaatgtccccggcctgtggtcaaatcgggagacaagcccagcctttcggcgagatacgtcagagccaaaagaggaagcggagagggcaggggaagtcttctaacatgcggggacgtggaggaaaatcccggccccatggccaccggcagcaggaccagcctgctgctggccttcggcctgctgtgcctgccctggctgcaggagggcagcgccgatgctagagtcacccagacaccaagggacaaggtgacagagatgggacaagaagtaacaatgagatgtcagccaattttaggccacaatactgttttctggtacagacagaccatgatgcaaggactggagttgctggcttacttccgcaaccgggctcctctagatgattcggggatgccgaaggatcgattctcagcagagatgcctgatgcaactttagccactctgaagatccagccctcagaacccagggactcagctgtgtatttttgtgctagtggtcccgaggggttggacaatgagcagttcttcgggccagggacacggctcaccgtgctagaggacctgaaaaacgtgttcccacccgaggtcgctgtgtttgagccatcagaagcagagatctcccacacccaaaaggccacactggtgtgcctggccacaggcttctaccccgaccacgtggagctgagctggtgggtgaatgggaaggaggtgcacagtggggtcagcacagacccgcagcccctcaaggagcagcccgccctcaatgactccagatactgcctgtcctcccgcctgagggtctcggccaccttctggcagaacccccgcaaccacttccgctgtcaagtccagttctacgggctctcggagaatgacgagtggacccaggatagggccaaacctgtcacccagatcgtcagcgccgaggcctggggtagagcagactgtggcttcacctccgagtcttaccagcaaggggtcctgtctgccaccatcctctatgagatcttgctagggaaggccaccttgtatgccgtgctggtcagtgccctcgtgctgatggccatggtcaagagaaaggattccagaggccgggccaagcggggatccggagccacaaatttctccctgctgaaacaggccggcgatgtggaggagaatcctggacctatggccaccggcagcaggaccagcctgctgctggccttcggcctgctgtgcctgccctggctgcaggagggcagcgcccagaaggaggtggagcagaattctggacccctcagtgttccagagggagccattgcctctctcaactgcacttacagtgaccgaggttcccagtccttcttctggtacagacaatattctgggaaaagccctgagttgataatgttcatatactccaatggtgacaaagaagatggaaggtttacagcacagctcaataaagccagccagtatgtttctctgctcatcagagactcccagcccagtgattcagccacctacctctgtgccgtgaacatgccaggcaacatgctcacctttggagggggaacaaggttaatggtcaaaccccat

SEQ ID NO: 396 - protein, 235 aa, synthetic construct
MALPVTALLLPLALLLHAARPSQFRVSPLDRTWNLGETVELKCQVLLSNPTSGCSWLFQPRGAAASPTFLLYLSQNKPKAAEGLDTQRFSGKRLGDTFVLTLSDFRRENEGYYFCSALSNSIMYFSHFVPVFLPAKPTTTPAPRPPTPAPTIASQPLSLRPEACRPAAGGAVHTRGLDFACDIYIWAPLAGTCGVLLLSLVITLYCNHRNRRRVCKCPRPVVKSGDKPSLSARYV

SEQ ID NO: 397 - DNA, 705 bp, synthetic construct
  source 1..705: mol_type = other DNA
atggccttaccagtgaccgccttgctcctgccgctggccttgctgctccacgccgccaggccgagccagttccgggtgtcgccgctggatcggacctggaacctgggcgagacagtggagctgaagtgccaggtgctgctgtccaacccgacgtcgggctgctcgtggctcttccagccgcgcggcgccgccgccagtcccaccttcctcctatacctctcccaaaacaagcccaaggcggccgaggggctggacacccagcggttctcgggcaagaggttgggggacaccttcgtcctcaccctgagcgacttccgccgagagaacgagggctactatttctgctcggccctgagcaactccatcatgtacttcagccacttcgtgccggtcttcctgccagcgaagcccaccacgacgccagcgccgcgaccaccaacaccggcgcccaccatcgcgtcgcagcccctgtccctgcgcccagaggcgtgccggccagcggcggggggcgcagtgcacacgagggggctggacttcgcctgtgatatctacatctgggcgcccttggccgggacttgtggggtccttctcctgtcactggttatcaccctttactgcaaccacaggaaccgaagacgtgtttgcaaatgtccccggcctgtggtcaaatcgggagacaagcccagcctttcggcgagatacgtc

SEQ ID NO: 398 - protein, 1001 aa, synthetic construct
GSGATNFSLLKQAGDVEENPGPMALPVTALLLPLALLLHAARPSQFRVSPLDRTWNLGETVELKCQVLLSNPTSGCSWLFQPRGAAASPTFLLYLSQNKPKAAEGLDTQRFSGKRLGDTFVLTLSDFRRENEGYYFCSALSNSIMYFSHFVPVFLPAKPTTTPAPRPPTPAPTIASQPLSLRPEACRPAAGGAVHTRGLDFACDIYIWAPLAGTCGVLLLSLVITLYCNHRNRRRVCKCPRPVVKSGDKPSLSARYVRAKRGSGQCTNYALLKLAGDVESNPGPMRPRLWLLLAAQLTVLHGNSVLQQTPAYIKVQTNKMVMLSCEAKISLSNMRIYWLRQRQAPSSDSHHEFLALWDSAKGTIHGEEVEQEKIAVFRDASRFILNLTSVKPEDSGIYFCMIVGSPELTFGKGTQLSVVDFLPTTAQPTKKSTLKKRVCRLPRPETQKGPLCSPITLGLLVAGVLVLLVSLGVAIHLCCRRRRARLRFMKQFYKRAKRGSGEGRGSLLTCGDVEENPGPMATGSRTSLLLAFGLLCLPWLQEGSADARVTQTPRDKVTEMGQEVTMRCQPILGHNTVFWYRQTMMQGLELLAYFRNRAPLDDSGMPKDRFSAEMPDATLATLKIQPSEPRDSAVYFCASGPEGLDNEQFFGPGTRLTVLEDLKNVFPPEVAVFEPSEAEISHTQKATLVCLATGFYPDHVELSWWVNGKEVHSGVSTDPQPLKEQPALNDSRYCLSSRLRVSATFWQNPRNHFRCQVQFYGLSENDEWTQDRAKPVTQIVSAEAWGRADCGFTSESYQQGVLSATILYEILLGKATLYAVLVSALVLMAMVKRKDSRGRAKRGSGATNFSLLKQAGDVEENPGPMATGSRTSLLLAFGLLCLPWLQEGSAQKEVEQNSGPLSVPEGAIASLNCTYSDRGSQSFFWYRQYSGKSPELIMFIYSNGDKEDGRFTAQLNKASQYVSLLIRDSQPSDSATYLCAVNMPGNMLTFGGGTRLMVKPH

SEQ ID NO: 399 - DNA, 3003 bp, synthetic construct
  source 1..3003: mol_type = other DNA
ggcagcggcgccaccaacttcagcctgctgaagcaggccggcgacgtggaggagaaccccggccccatggccttaccagtgaccgccttgctcctgccgctggccttgctgctccacgccgccaggccgagccagttccgggtgtcgccgctggatcggacctggaacctgggcgagacagtggagctgaagtgccaggtgctgctgtccaacccgacgtcgggctgctcgtggctcttccagccgcgcggcgccgccgccagtcccaccttcctcctatacctctcccaaaacaagcccaaggcggccgaggggctggacacccagcggttctcgggcaagaggttgggggacaccttcgtcctcaccctgagcgacttccgccgagagaacgagggctactatttctgctcggccctgagcaactccatcatgtacttcagccacttcgtgccggtcttcctgccagcgaagcccaccacgacgccagcgccgcgaccaccaacaccggcgcccaccatcgcgtcgcagcccctgtccctgcgcccagaggcgtgccggccagcggcggggggcgcagtgcacacgagggggctggacttcgcctgtgatatctacatctgggcgcccttggccgggacttgtggggtccttctcctgtcactggttatcaccctttactgcaaccacaggaaccgaagacgtgtttgcaaatgtccccggcctgtggtcaaatcgggagacaagcccagcctttcggcgagatacgtcagagccaaaagaggaagcggacagtgtactaattatgctctcttgaaattggctggagatgttgagagcaacccaggtcccatgcggccgcggctgtggctcctcttggccgcgcagctgacagttctccatggcaactcagtcctccagcagacccctgcatacataaaggtgcaaaccaacaagatggtgatgctgtcctgcgaggctaaaatctccctcagtaacatgcgcatctactggctgagacagcgccaggcaccgagcagtgacagtcaccacgagttcctggccctctgggattccgcaaaagggactatccacggtgaagaggtggaacaggagaagatagctgtgtttcgggatgcaagccggttcattctcaatctcacaagcgtgaagccggaagacagtggcatctacttctgcatgatcgtcgggagccccgagctgaccttcgggaagggaactcagctgagtgtggttgatttccttcccaccactgcccagcccaccaagaagtccaccctcaagaagagagtgtgccggttacccaggccagagacccagaagggcccactttgtagccccatcacccttggcctgctggtggctggcgtcctggttctgctggtttccctgggagtggccatccacctgtgctgccggcggaggagagcccggcttcgtttcatgaaacaattttacaaaagagccaaaagaggaagcggagagggcaggggaagtcttctaacatgcggggacgtggaggaaaatcccggccccatggccaccggcagcaggaccagcctgctgctggccttcggcctgctgtgcctgccctggctgcaggagggcagcgccgatgctagagtcacccagacaccaagggacaaggtgacagagatgggacaagaagtaacaatgagatgtcagccaattttaggccacaatactgttttctggtacagacagaccatgatgcaaggactggagttgctggcttacttccgcaaccgggctcctctagatgattcggggatgccgaaggatcgattctcagcagagatgcctgatgcaactttagccactctgaagatccagccctcagaacccagggactcagctgtgtatttttgtgctagtggtcccgaggggttggacaatgagcagttcttcgggccagggacacggctcaccgtgctagaggacctgaaaaacgtgttcccacccgaggtcgctgtgtttgagccatcagaagcagagatctcccacacccaaaaggccacactggtgtgcctggccacaggcttctaccccgaccacgtggagctgagctggtgggtgaatgggaaggaggtgcacagtggggtcagcacagacccgcagcccctcaaggagcagcccgccctcaatgactccagatactgcctgtcctcccgcctgagggtctcggccaccttctggcagaacccccgcaaccacttccgctgtcaagtccagttctacgggctctcggagaatgacgagtggacccaggatagggccaaacctgtcacccagatcgtcagcgccgaggcctggggtagagcagactgtggcttcacctccgagtcttaccagcaaggggtcctgtctgccaccatcctctatgagatcttgctagggaaggccaccttgtatgccgtgctggtcagtgccctcgtgctgatggccatggtcaagagaaaggattccagaggccgggccaagcggggatccggagccacaaatttctccctgctgaaacaggccggcgatgtggaggagaatcctggacctatggccaccggcagcaggaccagcctgctgctggccttcggcctgctgtgcctgccctggctgcaggagggcagcgcccagaaggaggtggagcagaattctggacccctcagtgttccagagggagccattgcctctctcaactgcacttacagtgaccgaggttcccagtccttcttctggtacagacaatattctgggaaaagccctgagttgataatgttcatatactccaatggtgacaaagaagatggaaggtttacagcacagctcaataaagccagccagtatgtttctctgctcatcagagactcccagcccagtgattcagccacctacctctgtgccgtgaacatgccaggcaacatgctcacctttggagggggaacaaggttaatggtcaaaccccat

SEQ ID NO: 400 - protein, 210 aa, synthetic construct
MRPRLWLLLAAQLTVLHGNSVLQQTPAYIKVQTNKMVMLSCEAKISLSNMRIYWLRQRQAPSSDSHHEFLALWDSAKGTIHGEEVEQEKIAVFRDASRFILNLTSVKPEDSGIYFCMIVGSPELTFGKGTQLSVVDFLPTTAQPTKKSTLKKRVCRLPRPETQKGPLCSPITLGLLVAGVLVLLVSLGVAIHLCCRRRRARLRFMKQFYK

SEQ ID NO: 401 - DNA, 630 bp, synthetic construct
  source 1..630: mol_type = other DNA
atgcggccgcggctgtggctcctcttggccgcgcagctgacagttctccatggcaactcagtcctccagcagacccctgcatacataaaggtgcaaaccaacaagatggtgatgctgtcctgcgaggctaaaatctccctcagtaacatgcgcatctactggctgagacagcgccaggcaccgagcagtgacagtcaccacgagttcctggccctctgggattccgcaaaagggactatccacggtgaagaggtggaacaggagaagatagctgtgtttcgggatgcaagccggttcattctcaatctcacaagcgtgaagccggaagacagtggcatctacttctgcatgatcgtcgggagccccgagctgaccttcgggaagggaactcagctgagtgtggttgatttccttcccaccactgcccagcccaccaagaagtccaccctcaagaagagagtgtgccggttacccaggccagagacccagaagggcccactttgtagccccatcacccttggcctgctggtggctggcgtcctggttctgctggtttccctgggagtggccatccacctgtgctgccggcggaggagagcccggcttcgtttcatgaaacaattttacaaa

SEQ ID NO: 402 - protein, 22 aa, synthetic construct
GSGATNFSLLKQAGDVEENPGP

SEQ ID NO: 403 - protein, 26 aa, synthetic construct
MATGSRTSLLLAFGLLCLPWLQEGSA

SEQ ID NO: 404 - protein, 26 aa, synthetic construct
RAKRGSGATNFSLLKQAGDVEENPGP

SEQ ID NO: 405 - protein, 1368 aa, synthetic construct [sequence omitted]